European Patent Specification EP 3 891 170 B1, published July 31, 2024. Title: HIV VACCINE IMMUNOGENS. Applicant: THE ROCKEFELLER UNIVERSITY. The sequence listing filed with the application follows.

SEQUENCE LISTING (495 sequences)

SEQ ID NO: 1 - protein, 666 aa, Artificial Sequence
  Description of Artificial Sequence: Synthetic polypeptide
MDAMKRGLCCVLLLCGAVFVSPSQEIHARFRRGARAENLWVTVYYGVPVWKDAETTLFCASDAKAYETEKHNVWATHACVPTDPNPQEIHLENVTEEFNMWKNNMVEQMHTDIISLWDQSLKPCVKLTPLCVTLQCTNVTNNITDDMRGELKNCSFNMTTELRDKKQKVYSLFYRLDVVQINENQGNRSNNSNKEYRLINCNTSAITQACPKVSFEPIPIHYCAPAGFAILKCKDKKFNGTGPCPSVSTVQCTHGIKPWSTQLLLNGSLAEEEVMIRSENITNNAKNILVQFNTPVQINCTRPNNNTRKSIRIGPGQAFYATGDIIGDIRQAHCNVSKATWNETLGKWKQLRKHFGNNTIIRFANSSGGDLEVTTHSFNCGGEFFYCNTSGLFNSTWISNTSVQGSNSTGSNDSITLPCRIKQIINMWQRIGQAMYAPPIQGVIRCVSNITGLILTRDGGSTNSTTETFRPGGGDMRDNWRSELYKYKWKIEPLGVAPTRCKRRVVGRRRRRRAVGIGAVFLGFLGAAGSTMGAASMTLTVQARNLLSGIVQQQSNLLRAPEAQQHLLKLTVWGIKQLQARVLAVERYLRDQQLLGIWGCSGKLICCTNVPWNSSWSNRNLSEIWDNMTWLQWDKEISNYTQIIYGLLEESQNQQEKNEQDLLALD

SEQ ID NO: 2 - protein, 659 aa, Artificial Sequence
  Description of Artificial Sequence: Synthetic polypeptide
MDAMKRGLCCVLLLCGAVFVSPAGAGSNLWVTVYYGVPVWKDAETTLFCASDAKAYETEKHNVWATHACVPTDPNPQEIHLENVTEEFNMWKNNMVEQMHEDIISLWDQSLKPCVKLTPLCVTLQCTNYAPNLLSNMRGELKQCSFNMTTELRDKKQKVYSLFYRLDVVQINENQGNRSNNSNKEYRLINCNTSAITQACPKVSFEPIPIHYCAPAGFAILKCKDKKFNGTGPCPSVSTVQCTHGIKPVVSTQLLLNGSLAEEEVIIRSENITNNAKNILVQLNTPVQINCTRPNNNTVKSIRIGPGQAFYYFGDIIGDIRMAHCNVSKATWNETLGKVVKQLRKHFGNNTIIRFAQSSGGDLEVTTHSFNCGGEFFYCNTSGLFNSTWISNTSVQGSNSTGSNDSIVLPCRIKQIINMWQRIGQAMYAPPIQGVIRCVSNITGLILTRDGGSTNSTTETFRPGGGDMRDNWRSELYKYKVVKIEPLGVAPTRCKRRVVGRRRRRRAVGIGAVSLGFLGAAGSTMGAASMTLTVQARNLLSGIVQQQSNLLRAPEPQQHLLKDTHWGIKQLQARVLAVEHYLRDQQLLGIWGCSGKLICCTNVPWNSSWSNRNLSEIWDNMTWLQWDKEISNYTQIIYGLLEESQNQQEKNEQDLLALD

SEQ ID NO: 3 - DNA, 1980 bp, Artificial Sequence
  Description of Artificial Sequence: Synthetic polynucleotide
atggacgccatgaagaggggactttgctgtgttcttctgctgtgtggcgccgtgtttgttagccccgctggggccggatccaacctgtgggtcactgtgtattatggtgtgccagtgtggaaggatgcagagacaacactcttttgcgcctccgacgctaaagcatacgaaacggagaagcacaacgtgtgggcgacccatgcctgtgtccctacagaccctaaccctcaggaaattcatcttgaaaatgtcacagaagagtttaacatgtggaaaaacaacatggtggaacagatgcacgaggatatcatttccctgtgggaccagagtctgaaaccatgtgtcaaacttactcctctgtgcgtgactctccagtgtacaaactacgcacccaaccttttgagtaatatgcggggcgagctcaagcagtgcagtttcaatatgacaaccgaattgagagacaaaaaacagaaagtatactccctcttctaccggctggacgtggtgcagatcaatgagaaccaaggaaatagaagcaacaacagtaacaaggaataccggctcataaattgcaataccagcgctattacgcaggcttgccctaaggtgagctttgagccaatcccgatacattattgtgccccggcaggcttcgctatactgaaatgcaaggataagaagtttaatgggacaggcccttgccctagcgtttcaacggtccaatgtacccacgggatcaagcccgtagtgtctacacagctcctgctgaacggcagcctggccgaagaggaggtcataattaggagcgagaacataactaacaacgctaaaaacattctcgtccagctcaatacacctgtgcagatcaactgcacccggcccaacaacaacaccgtgaagtccattagaattggtccgggacaggcattttactacttcggagatataataggcgatatcagaatggcgcactgtaacgtgagcaaggccacctggaacgagaccctgggcaaggtggtcaaacagttgcgcaagcactttgggaacaacaccattattcggtttgcccagtcttccggcggcgaccttgaagtgaccactcatagcttcaactgtggaggggagtttttctattgcaatacatcaggcctgttcaactctacatggatctcaaataccagtgtccaggggtcaaattccaccggtagcaacgacagcatcgtcttgccttgtcgaatcaagcagatcattaatatgtggcagaggattggtcaggccatgtacgcacctccaatacagggagtcattcggtgcgtcagcaatattactggattgatcctcaccagagatggcgggagtaccaatagcactaccgaaactttccgcccaggaggaggcgacatgcgggataattggagatcagagctgtataagtataaggtggtgaaaattgaacccctgggagtggcgccaactagatgtaaacggcgagtggttggccggagacggcggcggagagcagtggggattggcgctgtctcactcggtttcctgggtgctgccggcagtacaatgggcgccgccagcatgacgctcacagtgcaggcccggaatcttcttagcggaattgtgcaacaacaaagcaatctgttgagagccccggaaccgcagcaacatctgttgaaggacacacattggggcatcaagcagctgcaagctcgggttctggctgttgagcattacctgagagaccaacagctgctgggcatatggggatgctcaggaaaactgatctgctgcaccaatgtcccatggaacagctcatggtcaaacaggaacctgagcgagatctgggataacatgacctggttgcagtgggacaaagaaattagcaattacacacagatcatctacggcctcctggaggaaagccagaatcagcaggagaaaaatgagcaggatctgcttgcccttgactga

SEQ ID NO: 4 - protein, 688 aa, Artificial Sequence
  Description of Artificial Sequence: Synthetic polypeptide
MDAMKRGLCCVLLLCGAVFVSPAGAGSNLWVTVYYGVPVWKDAETTLFCASDAKAYETEKHNVWATHACVPTDPNPQEIHLENVTEEFNMWKNNMVEQMHEDIISLWDQSLKPCVKLTPLCVTLQCTNYAPNLLSNMRGELKQCSFNMTTELRDKKQKVYSLFYRLDVVQINENQGNRSNNSNKEYRLINCNTSAITQACPKVSFEPIPIHYCAPAGFAILKCKDKKFNGTGPCPSVSTVQCTHGIKPVVSTQLLLNGSLAEEEVIIRSENITNNAKNILVQLNTPVQINCTRPNNNTVKSIRIGPGQAFYYFGDIIGDIRMAHCNVSKATWNETLGKVVKQLRKHFGNNTIIRFAQSSGGDLEVTTHSFNCGGEFFYCNTSGLFNSTWISNTSVQGSNSTGSNDSIVLPCRIKQIINMWQRIGQAMYAPPIQGVIRCVSNITGLILTRDGGSTNSTTETFRPGGGDMRDNWRSELYKYKVVKIEPLGVAPTRCKRRVVGRRRRRRAVGIGAVSLGFLGAAGSTMGAASMTLTVQARNLLSGIVQQQSNLLRAPEPQQHLLKDTHWGIKQLQARVLAVEHYLRDQQLLGIWGCSGKLICCTNVPWNSSWSNRNLSEIWDNMTWLQWDKEISNYTQIIYGLLEESQNQQEKNEQDLLALDGGGGSGGGSGGGSGSGAHIVMVDAYKPTK

SEQ ID NO: 5 - DNA, 2067 bp, Artificial Sequence
  Description of Artificial Sequence: Synthetic polynucleotide
atggacgccatgaagaggggactttgctgtgttcttctgctgtgtggcgccgtgtttgttagccccgctggggccggatccaacctgtgggtcactgtgtattatggtgtgccagtgtggaaggatgcagagacaacactcttttgcgcctccgacgctaaagcatacgaaacggagaagcacaacgtgtgggcgacccatgcctgtgtccctacagaccctaaccctcaggaaattcatcttgaaaatgtcacagaagagtttaacatgtggaaaaacaacatggtggaacagatgcacgaggatatcatttccctgtgggaccagagtctgaaaccatgtgtcaaacttactcctctgtgcgtgactctccagtgtacaaactacgcacccaaccttttgagtaatatgcggggcgagctcaagcagtgcagtttcaatatgacaaccgaattgagagacaaaaaacagaaagtatactccctcttctaccggctggacgtggtgcagatcaatgagaaccaaggaaatagaagcaacaacagtaacaaggaataccggctcataaattgcaataccagcgctattacgcaggcttgccctaaggtgagctttgagccaatcccgatacattattgtgccccggcaggcttcgctatactgaaatgcaaggataagaagtttaatgggacaggcccttgccctagcgtttcaacggtccaatgtacccacgggatcaagcccgtagtgtctacacagctcctgctgaacggcagcctggccgaagaggaggtcataattaggagcgagaacataactaacaacgctaaaaacattctcgtccagctcaatacacctgtgcagatcaactgcacccggcccaacaacaacaccgtgaagtccattagaattggtccgggacaggcattttactacttcggagatataataggcgatatcagaatggcgcactgtaacgtgagcaaggccacctggaacgagaccctgggcaaggtggtcaaacagttgcgcaagcactttgggaacaacaccattattcggtttgcccagtcttccggcggcgaccttgaagtgaccactcatagcttcaactgtggaggggagtttttctattgcaatacatcaggcctgttcaactctacatggatctcaaataccagtgtccaggggtcaaattccaccggtagcaacgacagcatcgtcttgccttgtcgaatcaagcagatcattaatatgtggcagaggattggtcaggccatgtacgcacctccaatacagggagtcattcggtgcgtcagcaatattactggattgatcctcaccagagatggcgggagtaccaatagcactaccgaaactttccgcccaggaggaggcgacatgcgggataattggagatcagagctgtataagtataaggtggtgaaaattgaacccctgggagtggcgccaactagatgtaaacggcgagtggttggccggagacggcggcggagagcagtggggattggcgctgtctcactcggtttcctgggtgctgccggcagtacaatgggcgccgccagcatgacgctcacagtgcaggcccggaatcttcttagcggaattgtgcaacaacaaagcaatctgttgagagccccggaaccgcagcaacatctgttgaaggacacacattggggcatcaagcagctgcaagctcgggttctggctgttgagcattacctgagagaccaacagctgctgggcatatggggatgctcaggaaaactgatctgctgcaccaatgtcccatggaacagctcatggtcaaacaggaacctgagcgagatctgggataacatgacctggttgcagtgggacaaagaaattagcaattacacacagatcatctacggcctcctggaggaaagccagaatcagcaggagaaaaatgagcaggatctgcttgcccttgacggtggaggcggttcaggcggcggatctggcggtgggagcggttcgggagcccatatagtgatggttgatgcctataaaccgaccaagtga

SEQ ID NO: 6 - protein, 659 aa, Artificial Sequence
  Description of Artificial Sequence: Synthetic polypeptide
MDAMKRGLCCVLLLCGAVFVSPAGAGSNLWVTVYYGVPVWKDAETTLFCASDAKAYETEKHNVWATHACVPTDPNPQEIHLENVTEEFNMWKNNMVEQMHEDIISLWDQSLKPCVKLTPLCVTLQCTNYAPNLLSNMRGELKQCSFNMTTELRDKKQKVYSLFYRLDVVQINENQGNRSNNSNKEYRLINCNTSAITQACPKVSFEPIPIHYCAPAGFAILKCKNKTFNGTGPCPNVSTVQCTHGIKPVVSTQLLLNGSLAEEEVIIRSENITNNAKNILVQLNTSVQINCTRPNNNTVKSIRIGPGQAFYYFGDIIGDIRMAHCNVSKATWNETLGNVSKQLRKHFGNNTIIRFAQSSGGDLEVTTHSFNCGGEFFYCNTSGLFNSTWISNTSVQGSNSTGSNDSIVLPCRIKQIINMWQRIGQAMYAPPIQGVIRCVSNITGLILTRDGGSTNSTTETFRPGGGDMRDNWRSELYKYKVVKIEPLGVAPTRCKRRVVGRRRRRRAVGIGAVSLGFLGAAGSTMGAASMTLTVQARNLLSGIVQQQSNLLRAPEPQQHLLKDTHWGIKQLQARVLAVEHYLRDQQLLGIWGCSGKLICCTNVPWNSSWSNRNLSEIWDNMTWLQWDKEISNYTQIIYGLLEESQNQQEKNEQDLLALD

SEQ ID NO: 7 - DNA, 1980 bp, Artificial Sequence
  Description of Artificial Sequence: Synthetic polynucleotide
atggacgccatgaagaggggactttgctgtgttcttctgctgtgtggcgccgtgtttgttagccccgctggggccggatccaacctgtgggtcactgtgtattatggtgtgccagtgtggaaggatgcagagacaacactcttttgcgcctccgacgctaaagcatacgaaacggagaagcacaacgtgtgggcgacccatgcctgtgtccctacagaccctaaccctcaggaaattcatcttgaaaatgtcacagaagagtttaacatgtggaaaaacaacatggtggaacagatgcacgaggatatcatttccctgtgggaccagagtctgaaaccatgtgtcaaacttactcctctgtgcgtgactctccagtgtacaaactacgcacccaaccttttgagtaatatgcggggcgagctcaagcagtgcagtttcaatatgacaaccgaattgagagacaaaaaacagaaagtatactccctcttctaccggctggacgtggtgcagatcaatgagaaccaaggaaatagaagcaacaacagtaacaaggaataccggctcataaattgcaataccagcgctattacgcaggcttgccctaaggtgagctttgagccaatcccgatacattattgtgccccggcaggcttcgctatactgaaatgcaagaataagacgtttaatgggacaggcccttgccctaacgtttcaacggtccaatgtacccacgggatcaagcccgtagtgtctacacagctcctgctgaacggcagcctggccgaagaggaggtcataattaggagcgagaacataactaacaacgctaaaaacattctcgtccagctcaatacaagtgtgcagatcaactgcacccggcccaacaacaacaccgtgaagtccattagaattggtccgggacaggcattttactacttcggagatataataggcgatatcagaatggcgcactgtaacgtgagcaaggccacctggaacgagaccctgggcaatgtgagcaaacagttgcgcaagcactttgggaacaacaccattattcggtttgcccagtcttccggcggcgaccttgaagtgaccactcatagcttcaactgtggaggggagtttttctattgcaatacatcaggcctgttcaactctacatggatctcaaataccagtgtccaggggtcaaattccaccggtagcaacgacagcatcgtcttgccttgtcgaatcaagcagatcattaatatgtggcagaggattggtcaggccatgtacgcacctccaatacagggagtcattcggtgcgtcagcaatattactggattgatcctcaccagagatggcgggagtaccaatagcactaccgaaactttccgcccaggaggaggcgacatgcgggataattggagatcagagctgtataagtataaggtggtgaaaattgaacccctgggagtggcgccaactagatgtaaacggcgagtggttggccggagacggcggcggagagcagtggggattggcgctgtctcactcggtttcctgggtgctgccggcagtacaatgggcgccgccagcatgacgctcacagtgcaggcccggaatcttcttagcggaattgtgcaacaacaaagcaatctgttgagagccccggaaccgcagcaacatctgttgaaggacacacattggggcatcaagcagctgcaagctcgggttctggctgttgagcattacctgagagaccaacagctgctgggcatatggggatgctcaggaaaactgatctgctgcaccaatgtcccatggaacagctcatggtcaaacaggaacctgagcgagatctgggataacatgacctggttgcagtgggacaaagaaattagcaattacacacagatcatctacggcctcctggaggaaagccagaatcagcaggagaaaaatgagcaggatctgcttgcccttgactga

SEQ ID NO: 8 - protein, 688 aa, Artificial Sequence
  Description of Artificial Sequence: Synthetic polypeptide
MDAMKRGLCCVLLLCGAVFVSPAGAGSNLWVTVYYGVPVWKDAETTLFCASDAKAYETEKHNVWATHACVPTDPNPQEIHLENVTEEFNMWKNNMVEQMHEDIISLWDQSLKPCVKLTPLCVTLQCTNYAPNLLSNMRGELKQCSFNMTTELRDKKQKVYSLFYRLDVVQINENQGNRSNNSNKEYRLINCNTSAITQACPKVSFEPIPIHYCAPAGFAILKCKNKTFNGTGPCPNVSTVQCTHGIKPVVSTQLLLNGSLAEEEVIIRSENITNNAKNILVQLNTSVQINCTRPNNNTVKSIRIGPGQAFYYFGDIIGDIRMAHCNVSKATWNETLGNVSKQLRKHFGNNTIIRFAQSSGGDLEVTTHSFNCGGEFFYCNTSGLFNSTWISNTSVQGSNSTGSNDSIVLPCRIKQIINMWQRIGQAMYAPPIQGVIRCVSNITGLILTRDGGSTNSTTETFRPGGGDMRDNWRSELYKYKVVKIEPLGVAPTRCKRRVVGRRRRRRAVGIGAVSLGFLGAAGSTMGAASMTLTVQARNLLSGIVQQQSNLLRAPEPQQHLLKDTHWGIKQLQARVLAVEHYLRDQQLLGIWGCSGKLICCTNVPWNSSWSNRNLSEIWDNMTWLQWDKEISNYTQIIYGLLEESQNQQEKNEQDLLALDGGGGSGGGSGGGSGSGAHIVMVDAYKPTK

SEQ ID NO: 9 - DNA, 2067 bp, Artificial Sequence
  Description of Artificial Sequence: Synthetic polynucleotide
atggacgccatgaagaggggactttgctgtgttcttctgctgtgtggcgccgtgtttgttagccccgctggggccggatccaacctgtgggtcactgtgtattatggtgtgccagtgtggaaggatgcagagacaacactcttttgcgcctccgacgctaaagcatacgaaacggagaagcacaacgtgtgggcgacccatgcctgtgtccctacagaccctaaccctcaggaaattcatcttgaaaatgtcacagaagagtttaacatgtggaaaaacaacatggtggaacagatgcacgaggatatcatttccctgtgggaccagagtctgaaaccatgtgtcaaacttactcctctgtgcgtgactctccagtgtacaaactacgcacccaaccttttgagtaatatgcggggcgagctcaagcagtgcagtttcaatatgacaaccgaattgagagacaaaaaacagaaagtatactccctcttctaccggctggacgtggtgcagatcaatgagaaccaaggaaatagaagcaacaacagtaacaaggaataccggctcataaattgcaataccagcgctattacgcaggcttgccctaaggtgagctttgagccaatcccgatacattattgtgccccggcaggcttcgctatactgaaatgcaagaataagacgtttaatgggacaggcccttgccctaacgtttcaacggtccaatgtacccacgggatcaagcccgtagtgtctacacagctcctgctgaacggcagcctggccgaagaggaggtcataattaggagcgagaacataactaacaacgctaaaaacattctcgtccagctcaatacaagtgtgcagatcaactgcacccggcccaacaacaacaccgtgaagtccattagaattggtccgggacaggcattttactacttcggagatataataggcgatatcagaatggcgcactgtaacgtgagcaaggccacctggaacgagaccctgggcaatgtgagcaaacagttgcgcaagcactttgggaacaacaccattattcggtttgcccagtcttccggcggcgaccttgaagtgaccactcatagcttcaactgtggaggggagtttttctattgcaatacatcaggcctgttcaactctacatggatctcaaataccagtgtccaggggtcaaattccaccggtagcaacgacagcatcgtcttgccttgtcgaatcaagcagatcattaatatgtggcagaggattggtcaggccatgtacgcacctccaatacagggagtcattcggtgcgtcagcaatattactggattgatcctcaccagagatggcgggagtaccaatagcactaccgaaactttccgcccaggaggaggcgacatgcgggataattggagatcagagctgtataagtataaggtggtgaaaattgaacccctgggagtggcgccaactagatgtaaacggcgagtggttggccggagacggcggcggagagcagtggggattggcgctgtctcactcggtttcctgggtgctgccggcagtacaatgggcgccgccagcatgacgctcacagtgcaggcccggaatcttcttagcggaattgtgcaacaacaaagcaatctgttgagagccccggaaccgcagcaacatctgttgaaggacacacattggggcatcaagcagctgcaagctcgggttctggctgttgagcattacctgagagaccaacagctgctgggcatatggggatgctcaggaaaactgatctgctgcaccaatgtcccatggaacagctcatggtcaaacaggaacctgagcgagatctgggataacatgacctggttgcagtgggacaaagaaattagcaattacacacagatcatctacggcctcctggaggaaagccagaatcagcaggagaaaaatgagcaggatctgcttgcccttgacggtggaggcggttcaggcggcggatctggcggtgggagcggttcgggagcccatatagtgatggttgatgcctataaaccgaccaagtga

SEQ ID NO: 10 - protein, 45 aa, Human immunodeficiency virus
KGKGKGKGKGCTRPNNNTRKSIRIGPGQTFYATGDIIGDIRQAHC

SEQ ID NO: 11 - protein, 659 aa, Artificial Sequence
  Description of Artificial Sequence: Synthetic polypeptide
MDAMKRGLCCVLLLCGAVFVSPAGAGSNLWVTVYYGVPVWKDAETTLFCASDAKAYETEKHNVWATHACVPTDPNPQEIHLENVTEEFNMWKNNMVEQMHEDIISLWDQSLKPCVKLTPLCVTLQCTNYAPNLLSNMRGELKQCSFNMTTELRDKKQKVYSLFYRLDVVQINENQGNRSNNSNKEYRLINCNTSAITQACPKVSFEPIPIHYCAPAGFAILKCKNKTFNGTGPCPNVSTVQCTHGIKPVVSTQLLLNGSLAEEEVIIRSENITNNAKNILVQLNTPVQINCTRPNNNTVKSIRIGPGQAFYYFGDIIGDIRMAHCNVSKATWNETLGNVSKQLRKHFGNNTIIRFAQSSGGDLEVTTHSFNCGGEFFYCNTSGLFNSTWISNTSVQGSNSTGSNDSIVLPCRIKQIINMWQRIGQAMYAPPIQGVIRCVSNITGLILTRDGGSTNSTTETFRPGGGDMRDNWRSELYKYKVVKIEPLGVAPTRCKRRVVGRRRRRRAVGIGAVSLGFLGAAGSTMGAASMTLTVQARNLLSGIVQQQSNLLRAPEPQQHLLKDTHWGIKQLQARVLAVEHYLRDQQLLGIWGCSGKLICCTNVPWNSSWSNRNLSEIWDNMTWLQWDKEISNYTQIIYGLLEESQNQQEKNEQDLLALD

SEQ ID NO: 12 - DNA, 1980 bp, Artificial Sequence
  Description of Artificial Sequence: Synthetic polynucleotide
atggacgccatgaagaggggactttgctgtgttcttctgctgtgtggcgccgtgtttgttagccccgctggggccggatccaacctgtgggtcactgtgtattatggtgtgccagtgtggaaggatgcagagacaacactcttttgcgcctccgacgctaaagcatacgaaacggagaagcacaacgtgtgggcgacccatgcctgtgtccctacagaccctaaccctcaggaaattcatcttgaaaatgtcacagaagagtttaacatgtggaaaaacaacatggtggaacagatgcacgaggatatcatttccctgtgggaccagagtctgaaaccatgtgtcaaacttactcctctgtgcgtgactctccagtgtacaaactacgcacccaaccttttgagtaatatgcggggcgagctcaagcagtgcagtttcaatatgacaaccgaattgagagacaaaaaacagaaagtatactccctcttctaccggctggacgtggtgcagatcaatgagaaccaaggaaatagaagcaacaacagtaacaaggaataccggctcataaattgcaataccagcgctattacgcaggcttgccctaaggtgagctttgagccaatcccgatacattattgtgccccggcaggcttcgctatactgaaatgcaagaataagacgtttaatgggacaggcccttgccctaacgtttcaacggtccaatgtacccacgggatcaagcccgtagtgtctacacagctcctgctgaacggcagcctggccgaagaggaggtcataattaggagcgagaacataactaacaacgctaaaaacattctcgtccagctcaatacacctgtgcagatcaactgcacccggcccaacaacaacaccgtgaagtccattagaattggtccgggacaggcattttactacttcggagatataataggcgatatcagaatggcgcactgtaacgtgagcaaggccacctggaacgagaccctgggcaatgtgagcaaacagttgcgcaagcactttgggaacaacaccattattcggtttgcccagtcttccggcggcgaccttgaagtgaccactcatagcttcaactgtggaggggagtttttctattgcaatacatcaggcctgttcaactctacatggatctcaaataccagtgtccaggggtcaaattccaccggtagcaacgacagcatcgtcttgccttgtcgaatcaagcagatcattaatatgtggcagaggattggtcaggccatgtacgcacctccaatacagggagtcattcggtgcgtcagcaatattactggattgatcctcaccagagatggcgggagtaccaatagcactaccgaaactttccgcccaggaggaggcgacatgcgggataattggagatcagagctgtataagtataaggtggtgaaaattgaacccctgggagtggcgccaactagatgtaaacggcgagtggttggccggagacggcggcggagagcagtggggattggcgctgtctcactcggtttcctgggtgctgccggcagtacaatgggcgccgccagcatgacgctcacagtgcaggcccggaatcttcttagcggaattgtgcaacaacaaagcaatctgttgagagccccggaaccgcagcaacatctgttgaaggacacacattggggcatcaagcagctgcaagctcgggttctggctgttgagcattacctgagagaccaacagctgctgggcatatggggatgctcaggaaaactgatctgctgcaccaatgtcccatggaacagctcatggtcaaacaggaacctgagcgagatctgggataacatgacctggttgcagtgggacaaagaaattagcaattacacacagatcatctacggcctcctggaggaaagccagaatcagcaggagaaaaatgagcaggatctgcttgcccttgactga

SEQ ID NO: 13 - protein, 688 aa, Artificial Sequence
  Description of Artificial Sequence: Synthetic polypeptide
MDAMKRGLCCVLLLCGAVFVSPAGAGSNLWVTVYYGVPVWKDAETTLFCASDAKAYETEKHNVWATHACVPTDPNPQEIHLENVTEEFNMWKNNMVEQMHEDIISLWDQSLKPCVKLTPLCVTLQCTNYAPNLLSNMRGELKQCSFNMTTELRDKKQKVYSLFYRLDVVQINENQGNRSNNSNKEYRLINCNTSAITQACPKVSFEPIPIHYCAPAGFAILKCKNKTFNGTGPCPNVSTVQCTHGIKPVVSTQLLLNGSLAEEEVIIRSENITNNAKNILVQLNTPVQINCTRPNNNTVKSIRIGPGQAFYYFGDIIGDIRMAHCNVSKATWNETLGNVSKQLRKHFGNNTIIRFAQSSGGDLEVTTHSFNCGGEFFYCNTSGLFNSTWISNTSVQGSNSTGSNDSIVLPCRIKQIINMWQRIGQAMYAPPIQGVIRCVSNITGLILTRDGGSTNSTTETFRPGGGDMRDNWRSELYKYKVVKIEPLGVAPTRCKRRVVGRRRRRRAVGIGAVSLGFLGAAGSTMGAASMTLTVQARNLLSGIVQQQSNLLRAPEPQQHLLKDTHWGIKQLQARVLAVEHYLRDQQLLGIWGCSGKLICCTNVPWNSSWSNRNLSEIWDNMTWLQWDKEISNYTQIIYGLLEESQNQQEKNEQDLLALDGGGGSGGGSGGGSGSGAHIVMVDAYKPTK

SEQ ID NO: 14 - DNA, 2067 bp, Artificial Sequence
  Description of Artificial Sequence: Synthetic polynucleotide
atggacgccatgaagaggggactttgctgtgttcttctgctgtgtggcgccgtgtttgttagccccgctggggccggatccaacctgtgggtcactgtgtattatggtgtgccagtgtggaaggatgcagagacaacactcttttgcgcctccgacgctaaagcatacgaaacggagaagcacaacgtgtgggcgacccatgcctgtgtccctacagaccctaaccctcaggaaattcatcttgaaaatgtcacagaagagtttaacatgtggaaaaacaacatggtggaacagatgcacgaggatatcatttccctgtgggaccagagtctgaaaccatgtgtcaaacttactcctctgtgcgtgactctccagtgtacaaactacgcacccaaccttttgagtaatatgcggggcgagctcaagcagtgcagtttcaatatgacaaccgaattgagagacaaaaaacagaaagtatactccctcttctaccggctggacgtggtgcagatcaatgagaaccaaggaaatagaagcaacaacagtaacaaggaataccggctcataaattgcaataccagcgctattacgcaggcttgccctaaggtgagctttgagccaatcccgatacattattgtgccccggcaggcttcgctatactgaaatgcaagaataagacgtttaatgggacaggcccttgccctaacgtttcaacggtccaatgtacccacgggatcaagcccgtagtgtctacacagctcctgctgaacggcagcctggccgaagaggaggtcataattaggagcgagaacataactaacaacgctaaaaacattctcgtccagctcaatacacctgtgcagatcaactgcacccggcccaacaacaacaccgtgaagtccattagaattggtccgggacaggcattttactacttcggagatataataggcgatatcagaatggcgcactgtaacgtgagcaaggccacctggaacgagaccctgggcaatgtgagcaaacagttgcgcaagcactttgggaacaacaccattattcggtttgcccagtcttccggcggcgaccttgaagtgaccactcatagcttcaactgtggaggggagtttttctattgcaatacatcaggcctgttcaactctacatggatctcaaataccagtgtccaggggtcaaattccaccggtagcaacgacagcatcgtcttgccttgtcgaatcaagcagatcattaatatgtggcagaggattggtcaggccatgtacgcacctccaatacagggagtcattcggtgcgtcagcaatattactggattgatcctcaccagagatggcgggagtaccaatagcactaccgaaactttccgcccaggaggaggcgacatgcgggataattggagatcagagctgtataagtataaggtggtgaaaattgaacccctgggagtggcgccaactagatgtaaacggcgagtggttggccggagacggcggcggagagcagtggggattggcgctgtctcactcggtttcctgggtgctgccggcagtacaatgggcgccgccagcatgacgctcacagtgcaggcccggaatcttcttagcggaattgtgcaacaacaaagcaatctgttgagagccccggaaccgcagcaacatctgttgaaggacacacattggggcatcaagcagctgcaagctcgggttctggctgttgagcattacctgagagaccaacagctgctgggcatatggggatgctcaggaaaactgatctgctgcaccaatgtcccatggaacagctcatggtcaaacaggaacctgagcgagatctgggataacatgacctggttgcagtgggacaaagaaattagcaattacacacagatcatctacggcctcctggaggaaagccagaatcagcaggagaaaaatgagcaggatctgcttgcccttgacggtggaggcggttcaggcggcggatctggcggtgggagcggttcgggagcccatatagtgatggttgatgcctataaaccgaccaagtga

SEQ ID NO: 15 - protein, 4 aa, Human immunodeficiency virus
GDIR

SEQ ID NO: 16 - protein, 4 aa, Artificial Sequence
  Description of Artificial Sequence: Synthetic peptide
GAIA

SEQ ID NO: 17 - protein, 4 aa, Human immunodeficiency virus
REKR

SEQ ID NO: 18 - protein, 6 aa, Artificial Sequence
  Description of Artificial Sequence: Synthetic peptide
RRRRRR

SEQ ID NO: 19 - protein, 6 aa, Artificial Sequence
  Description of Artificial Sequence: Synthetic 6xHis tag
HHHHHH

SEQ ID NO: 20 - protein, 6 aa, Artificial Sequence
  Description of Artificial Sequence: Synthetic peptide
  MOD_RES (2)..(3): Any amino acid
QXXDSS

SEQ ID NO: 21 - protein, 4 aa, Artificial Sequence
  Description of Artificial Sequence: Synthetic peptide
SYAG

SEQ ID NO: 22 - protein, 11 aa, Artificial Sequence
  Description of Artificial Sequence: Synthetic peptide
ASGDELAWFAY

SEQ ID NO: 23 - protein, 11 aa, Artificial Sequence
  Description of Artificial Sequence: Synthetic peptide
ASGDELACFAY

SEQ ID NO: 24 - protein, 11 aa, Artificial Sequence
  Description of Artificial Sequence: Synthetic peptide
ANGDALAWFAY

SEQ ID NO: 25 - protein, 11 aa, Artificial Sequence
  Description of Artificial Sequence: Synthetic peptide
ACGDELAWFAY

SEQ ID NO: 26 - protein, 11 aa, Artificial Sequence
  Description of Artificial Sequence: Synthetic peptide
AGGDELAWFAY

SEQ ID NO: 27 - protein, 14 aa, Artificial Sequence
  Description of Artificial Sequence: Synthetic peptide
VRGEVYYDYDGFAY

SEQ ID NO: 28 - protein, 14 aa, Artificial Sequence
  Description of Artificial Sequence: Synthetic peptide
ARGEVYYDYDGFAY

SEQ ID NO: 29 - protein, 16 aa, Artificial Sequence
  Description of Artificial Sequence: Synthetic peptide
ARIRSDYDVGWWYFDV

SEQ ID NO: 30 - protein, 11 aa, Artificial Sequence
  Description of Artificial Sequence: Synthetic peptide
ARYYYGHYFDY

SEQ ID NO: 31 - protein, 10 aa, Artificial Sequence
  Description of Artificial Sequence: Synthetic peptide
VRSGIYYFDY

SEQ ID NO: 32 - protein, 11 aa, Artificial Sequence
  Description of Artificial Sequence: Synthetic peptide
ARYLLLRPFDY

SEQ ID NO: 33 - protein, 12 aa, Artificial Sequence
  Description of Artificial Sequence: Synthetic peptide
ARAGTTGYVMDY

SEQ ID NO: 34 - protein, 11 aa, Artificial Sequence
  Description of Artificial Sequence: Synthetic peptide
AIASYYYTLDY

SEQ ID NO: 35 - protein, 12 aa, Artificial Sequence
  Description of Artificial Sequence: Synthetic peptide
ARRGAAQAPFAY

SEQ ID NO: 36 - protein, 11 aa, Artificial Sequence
  Description of Artificial Sequence: Synthetic peptide
VRSELGPAFAY

SEQ ID NO: 37 - protein, 12 aa, Artificial Sequence
  Description of Artificial Sequence: Synthetic peptide
ARRGYGYGAMDY

SEQ ID NO: 38 - protein, 13 aa, Artificial Sequence
  Description of Artificial Sequence: Synthetic peptide
ARAYSNYVPWFAY

SEQ ID NO: 39 - protein, 10 aa, Artificial Sequence
  Description of Artificial Sequence: Synthetic peptide
ARREYGFFDY

SEQ ID NO: 40 - protein, 14 aa, Artificial Sequence
  Description of Artificial Sequence: Synthetic peptide
ARHGRLTGTGAMDY

SEQ ID NO: 41 - protein, 11 aa, Artificial Sequence
  Description of Artificial Sequence: Synthetic peptide
ARHGAGNALDY

SEQ ID NO: 42 - protein, 11 aa, Artificial Sequence
  Description of Artificial Sequence: Synthetic peptide
ARHGAGNAMDY

SEQ ID NO: 43 - protein, 9 aa, Artificial Sequence
  Description of Artificial Sequence: Synthetic peptide
QVEVTMWTT

SEQ ID NO: 44 - protein, 9 aa, Artificial Sequence
  Description of Artificial Sequence: Synthetic peptide
ASGRNYVDY

SEQ ID NO: 45 - protein, 9 aa, Artificial Sequence
  Description of Artificial Sequence: Synthetic peptide
ASGPNYFDY

SEQ ID NO: 46 - protein, 15 aa, Artificial Sequence
  Description of Artificial Sequence: Synthetic peptide
ARHGHYYGSSYGMDY

SEQ ID NO: 47 - protein, 12 aa, Artificial Sequence
  Description of Artificial Sequence: Synthetic peptide
ARDDGGYWYFDV

SEQ ID NO: 48 - protein, 12 aa, Artificial Sequence
  Description of Artificial Sequence: Synthetic peptide
ANIPKDRLCYGP

SEQ ID NO: 49 - protein, 12 aa, Artificial Sequence
  Description of Artificial Sequence: Synthetic peptide
ARHEEDGYWFAY

SEQ ID NO: 50 - protein, 9 aa, Artificial Sequence
  Description of Artificial Sequence: Synthetic peptide
LQYDEFPYT

SEQ ID NO: 51 - protein, 9 aa, Artificial Sequence
  Description of Artificial Sequence: Synthetic peptide
LHYDDFPYT

SEQ ID NO: 52 - protein, 9 aa, Artificial Sequence
  Description of Artificial Sequence: Synthetic peptide
LQYDEFPFT

SEQ ID NO: 53 - protein, 9 aa, Artificial Sequence
  Description of Artificial Sequence: Synthetic peptide
LRYDDFPYT

SEQ ID NO: 54 - protein, 9 aa, Artificial Sequence
  Description of Artificial Sequence: Synthetic peptide
IQYDEFPYT

SEQ ID NO: 55 - protein, 9 aa, Artificial Sequence
  Description of Artificial Sequence: Synthetic peptide
LHYDEFPYT

SEQ ID NO: 56 - protein, 9 aa, Artificial Sequence
  Description of Artificial Sequence: Synthetic peptide
LHYDDLPYT

SEQ ID NO: 57 - protein, 9 aa, Artificial Sequence
  Description of Artificial Sequence: Synthetic peptide
LQYDEFPHT

SEQ ID NO: 58 - protein, 9 aa, Artificial Sequence
  Description of Artificial Sequence: Synthetic peptide
LQYDESPYT

SEQ ID NO: 59 - protein, 9 aa, Artificial Sequence
  Description of Artificial Sequence: Synthetic peptide
LQYDEFPCT

SEQ ID NO: 60 - protein, 9 aa, Artificial Sequence
  Description of Artificial Sequence: Synthetic peptide
LQYDDFPHT

SEQ ID NO: 61 - protein, 9 aa, Artificial Sequence
  Description of Artificial Sequence: Synthetic peptide
QQSNEDPYT

SEQ ID NO: 62 - protein, 9 aa, Artificial Sequence
  Description of Artificial Sequence: Synthetic peptide
QQSNVDPYT

SEQ ID NO: 63 - protein, 9 aa, Artificial Sequence
  Description of Artificial Sequence: Synthetic peptide
QQSHEDPYT

SEQ ID NO: 64 - protein, 9 aa, Artificial Sequence
  Description of Artificial Sequence: Synthetic peptide
QHSNEDPYT

SEQ ID NO: 65 - protein, 10 aa, Artificial Sequence
  Description of Artificial Sequence: Synthetic peptide
QQSNEDPPWT

SEQ ID NO: 66 - protein, 10 aa, Artificial Sequence
  Description of Artificial Sequence: Synthetic peptide
QQGNEDPPWT

SEQ ID NO: 67 - protein, 10 aa, Artificial Sequence
  Description of Artificial Sequence: Synthetic peptide
HQSNEDPPWT

SEQ ID NO: 68 - protein, 10 aa, Artificial Sequence
  Description of Artificial Sequence: Synthetic peptide
QQINEDPPWT

SEQ ID NO: 69 - protein, 10 aa, Artificial Sequence
  Description of Artificial Sequence: Synthetic peptide
QQSYEDPPWT

SEQ ID NO: 70 - protein, 9 aa, Artificial Sequence
  Description of Artificial Sequence: Synthetic peptide
QQSNEDPWT

SEQ ID NO: 71 - protein, 9 aa, Artificial Sequence
  Description of Artificial Sequence: Synthetic peptide
QQNNEDPWT

SEQ ID NO: 72 - protein, 9 aa, Artificial Sequence
  Description of Artificial Sequence: Synthetic peptide
LQYDEFTFT

SEQ ID NO: 73 - protein, 9 aa, Artificial Sequence
  Description of Artificial Sequence: Synthetic peptide
QQYDSYPYT

SEQ ID NO: 74 - protein, 9 aa, Artificial Sequence
  Description of Artificial Sequence: Synthetic peptide
QQYNNYPYT

SEQ ID NO: 75 - protein, 9 aa, Artificial Sequence
  Description of Artificial Sequence: Synthetic peptide
QQYNSYPYT

SEQ ID NO: 76 - protein, 9 aa, Artificial Sequence
  Description of Artificial Sequence: Synthetic peptide
QQYNTYPYT

SEQ ID NO: 77 - protein, 9 aa, Artificial Sequence
  Description of Artificial Sequence: Synthetic peptide
QQYNIYPYT

SEQ ID NO: 78 - protein, 9 aa, Artificial Sequence
  Description of Artificial Sequence: Synthetic peptide
QQSNEDPFT

SEQ ID NO: 79 - protein, 9 aa, Artificial Sequence
  Description of Artificial Sequence: Synthetic peptide
LQYDEYMYT

SEQ ID NO: 80 - protein, 9 aa, Artificial Sequence
  Description of Artificial Sequence: Synthetic peptide
QQGNTLPWT

SEQ ID NO: 81 - protein, 9 aa, Artificial Sequence
  Description of Artificial Sequence: Synthetic peptide
QQGNTIPWT

SEQ ID NO: 82 - protein, 9 aa, Artificial Sequence
  Description of Artificial Sequence: Synthetic peptide
QQGNTLPRT

SEQ ID NO: 83 - protein, 8 aa, Artificial Sequence
  Description of Artificial Sequence: Synthetic peptide
SQSTHVPT

SEQ ID NO: 84 - protein, 9 aa, Artificial Sequence
  Description of Artificial Sequence: Synthetic peptide
VQYVQFPLT

SEQ ID NO: 85 - protein, 9 aa, Artificial Sequence
  Description of Artificial Sequence: Synthetic peptide
VQYAQFPLT

SEQ ID NO: 86 - protein, 9 aa, Artificial Sequence
  Description of Artificial Sequence: Synthetic peptide
FQGSHVPWT

SEQ ID NO: 87 - protein, 9 aa, Artificial Sequence
  Description of Artificial Sequence: Synthetic peptide
VQYAQFPFT

SEQ ID NO: 88 - protein, 9 aa, Artificial Sequence
  Description of Artificial Sequence: Synthetic peptide
LQHGESPYT

SEQ ID NO: 89 - protein, 9 aa, Artificial Sequence
  Description of Artificial Sequence: Synthetic peptide
QQFTSSPYT

SEQ ID NO: 90 - protein, 9 aa, Artificial Sequence
  Description of Artificial Sequence: Synthetic peptide
QQGNTLPYT

SEQ ID NO: 91 - protein, 9 aa, Artificial Sequence
  Description of Artificial Sequence: Synthetic peptide
LQYDEFRTT

SEQ ID NO: 92 - protein, 9 aa, Artificial Sequence
  Description of Artificial Sequence: Synthetic peptide
QQYNSYPFT

SEQ ID NO: 93 - protein, 9 aa, Artificial Sequence
  Description of Artificial Sequence: Synthetic peptide
QQCSGYPLT

SEQ ID NO: 94 - protein, 9 aa, Artificial Sequence
  Description of Artificial Sequence: Synthetic peptide
QQYSKLPWT

SEQ ID NO: 95 - protein, 10 aa, Artificial Sequence
  Description of Artificial Sequence: Synthetic peptide
LQYDEFPPFT

SEQ ID NO: 96 - protein, 13 aa, Artificial Sequence
  Description of Artificial Sequence: Synthetic peptide
ARHSRTGTGAMDY

SEQ ID NO: 97 - protein, 14 aa, Artificial Sequence
  Description of Artificial Sequence: Synthetic peptide
ARPYYYGSSPYFDY

SEQ ID NO: 98 - protein, 8 aa, Artificial Sequence
  Description of Artificial Sequence: Synthetic peptide
ARSIVPDY

SEQ ID NO: 99 - protein, 10 aa, Artificial Sequence
  Description of Artificial Sequence: Synthetic peptide
ASLYGNAFDY

SEQ ID NO: 100 - protein, 9 aa, Artificial Sequence
  Description of Artificial Sequence: Synthetic peptide
ASGGNYFDY

SEQ ID NO: 101 - protein, 11 aa, Artificial Sequence
  Description of Artificial Sequence: Synthetic peptide
ARHVGDHAMDY

SEQ ID NO: 102 - protein, 14 aa, Artificial Sequence
  Description of Artificial Sequence: Synthetic peptide
ARPYYYGSSPNFDY

SEQ ID NO: 103 - protein, 9 aa, Artificial Sequence
  Description of Artificial Sequence: Synthetic peptide
GTGKNYFDH

SEQ ID NO: 104 - protein, 10 aa, Artificial Sequence
  Description of Artificial Sequence: Synthetic peptide
ATNYGAWFPY

SEQ ID NO: 105 - protein, 14 aa, Artificial Sequence
  Description of Artificial Sequence: Synthetic peptide
ARHGITTVGVAMDY

SEQ ID NO: 106 - protein, 11 aa, Artificial Sequence
  Description of Artificial Sequence: Synthetic peptide
ANIPKDRLCYG

SEQ ID NO: 107 - protein, 13 aa, Artificial Sequence
  Description of Artificial Sequence: Synthetic peptide
ARHEGNYLYAMDY

SEQ ID NO: 108 - protein, 15 aa, Artificial Sequence
  Description of Artificial Sequence: Synthetic peptide
ARPPFITVVANYFDY

SEQ ID NO: 109 - protein, 9 aa, Artificial Sequence
  Description of Artificial Sequence: Synthetic peptide
QQRSSYPPT

SEQ ID NO: 110 - protein, 11 aa, Artificial Sequence
  Description of Artificial Sequence: Synthetic peptide
ARVVNYGPLDY

SEQ ID NO: 111 - protein, 11 aa, Artificial Sequence
  Description of Artificial Sequence: Synthetic peptide
ARVVKNGPLDY

SEQ ID NO: 112 - protein, 11 aa, Artificial Sequence
  Description of Artificial Sequence: Synthetic peptide
ARVVKYGPLDY

SEQ ID NO: 113 - protein, 11 aa, Artificial Sequence
  Description of Artificial Sequence: Synthetic peptide
ARLVRYGPLDY

SEQ ID NO: 114 - protein, 11 aa, Artificial Sequence
  Description of Artificial Sequence: Synthetic peptide
ARIVKYGPLDF

SEQ ID NO: 115 - protein, 11 aa, Artificial Sequence
  Description of Artificial Sequence: Synthetic peptide
ARGSRIAPFDY

SEQ ID NO: 116 - protein, 11 aa, Artificial Sequence
  Description of Artificial Sequence: Synthetic peptide
ARGSRIAPFDH

SEQ ID NO: 117 - protein, 11 aa, Artificial Sequence
  Description of Artificial Sequence: Synthetic peptide
SRYQARGPIDS

SEQ ID NO: 118 - protein, 11 aa, Artificial Sequence
  Description of Artificial Sequence: Synthetic peptide
ARDQARGPIDY

SEQ ID NO: 119 - protein, 11 aa, Artificial Sequence
  Description of Artificial Sequence: Synthetic peptide
ARNQARGPIDY

SEQ ID NO: 120 - protein, 11 aa, Artificial Sequence
  Description of Artificial Sequence: Synthetic peptide
ARDNRIGPFDY

SEQ ID NO: 121 - protein, 11 aa, Artificial Sequence
  Description of Artificial Sequence: Synthetic peptide
ARDKRIGPFDY

SEQ ID NO: 122 - protein, 11 aa, Artificial Sequence
  Description of Artificial Sequence: Synthetic peptide
AKKRRQLENDY

SEQ ID NO: 123 - protein, 11 aa, Artificial Sequence
  Description of Artificial Sequence: Synthetic peptide
VKKRRQLENDY

SEQ ID NO: 124 - protein, 11 aa, Artificial Sequence
  Description of Artificial Sequence: Synthetic peptide
ASRIAGGPFDY

SEQ ID NO: 125 - protein, 11 aa, Artificial Sequence
  Description of Artificial Sequence: Synthetic peptide
ASRIAGGPFDF

SEQ ID NO: 126 - protein, 11 aa, Artificial Sequence
  Description of Artificial Sequence: Synthetic peptide
ASLIAAGPFDY

SEQ ID NO: 127 - protein, 11 aa, Artificial Sequence
  Description of Artificial Sequence: Synthetic peptide
ASRIRGGPFDY

SEQ ID NO: 128 - protein, 11 aa, Artificial Sequence
  Description of Artificial Sequence: Synthetic peptide
ARDIVVGPIDY

SEQ ID NO: 129 - protein, 11 aa, Artificial Sequence
  Description of Artificial Sequence: Synthetic peptide
ARDIVIGPIDY

SEQ ID NO: 130 - protein, 11 aa, Artificial Sequence
  Description of Artificial Sequence: Synthetic peptide
ATVGRLAPFDY

SEQ ID NO: 131 - protein, 11 aa, Artificial Sequence
  Description of Artificial Sequence: Synthetic peptide
ARVGRVVPFDY

SEQ ID NO: 132 - protein, 11 aa, Artificial Sequence
  Description of Artificial Sequence: Synthetic peptide
ARVGRVAPFDY

SEQ ID NO: 133 - protein, 16 aa, Artificial Sequence
  Description of Artificial Sequence: Synthetic peptide
AKSPWGQSSSFEYFEF

SEQ ID NO: 134 - protein, 16 aa, Artificial Sequence
  Description of Artificial Sequence: Synthetic peptide
AKSPWGQSTSFEYFEF

SEQ ID NO: 135 - protein, 16 aa, Artificial Sequence
  Description of Artificial Sequence: Synthetic peptide
AKSPWGQSSYFEYFEF

SEQ ID NO: 136 - protein, 16 aa, Artificial Sequence
  Description of Artificial Sequence: Synthetic peptide
ASVLWGLPQDDNSLDV

SEQ ID NO: 137 - protein, 16 aa, Artificial Sequence
  Description of Artificial Sequence: Synthetic peptide
ASVLWEVPQDDNSLDV

SEQ ID NO: 138 - protein, 16 aa, Artificial Sequence
  Description of Artificial Sequence: Synthetic peptide
ANVLWGLPQDDNSLDV

SEQ ID NO: 139 - protein, 11 aa, Artificial Sequence
  Description of Artificial Sequence: Synthetic peptide
ASLQRLGPIDY

SEQ ID NO: 140 - protein, 11 aa, Artificial Sequence
  Description of Artificial Sequence: Synthetic peptide
ASLQYFGPFEF

SEQ ID NO: 141 - protein, 11 aa, Artificial Sequence
  Description of Artificial Sequence: Synthetic peptide
ASLQYFGPFDF

SEQ ID NO: 142 - protein, 11 aa, Artificial Sequence
  Description of Artificial Sequence: Synthetic peptide
ARAERAGPFDY

SEQ ID NO: 143 - protein, 11 aa, Artificial Sequence
  Description of Artificial Sequence: Synthetic peptide
ARHPHLESFDY

SEQ ID NO: 144 - protein, 12 aa, Artificial Sequence
  Description of Artificial Sequence: Synthetic peptide
ARNYGNYGYFEF

SEQ ID NO: 145 - protein, 16 aa, Artificial Sequence
  Description of Artificial Sequence: Synthetic peptide
ATGPYWGDYYGRYFEL

SEQ ID NO: 146 - protein, 16 aa, Artificial Sequence
  Description of Artificial Sequence: Synthetic peptide
ATGPYWGDYYGRYFEF

SEQ ID NO: 147 - protein, 11 aa, Artificial Sequence
  Description of Artificial Sequence: Synthetic peptide
ATERRAGPVDY

SEQ ID NO: 148 - protein, 11 aa, Artificial Sequence
  Description of Artificial Sequence: Synthetic peptide
ATDRRAGPLDY

SEQ ID NO: 149 - protein, 12 aa, Artificial Sequence
  Description of Artificial Sequence: Synthetic peptide
AGTLAGTTSFDV

SEQ ID NO: 150 - protein, 12 aa, Artificial Sequence
  Description of Artificial Sequence: Synthetic peptide
AGGLGRTTSFDV

SEQ ID NO: 151 - protein, 15 aa, Artificial Sequence
  Description of Artificial Sequence: Synthetic peptide
ARVGSGWSTEGNFDY

SEQ ID NO: 152 - protein, 16 aa, Artificial Sequence
  Description of Artificial Sequence: Synthetic peptide
AKDWIQWLHLGSYFDF

SEQ ID NO: 153 - protein, 16 aa, Artificial Sequence
  Description of Artificial Sequence: Synthetic peptide
AKDWIQWVHLGSYFDY

SEQ ID NO: 154 - protein, 13 aa, Artificial Sequence
  Description of Artificial Sequence: Synthetic peptide
ARHSSTYVAPVDY

SEQ ID NO: 155 - protein, 12 aa, Artificial Sequence
  Description of Artificial Sequence: Synthetic peptide
ASAKGRLAPLDY

SEQ ID NO: 156 - protein, 9 aa, Artificial Sequence
  Description of Artificial Sequence: Synthetic peptide
ANWADYFDY

SEQ ID NO: 157 - protein, 16 aa, Artificial Sequence
  Description of Artificial Sequence: Synthetic peptide
ARDPVITITTRERFDV

SEQ ID NO: 158 - protein, 11 aa, Artificial Sequence
  Description of Artificial Sequence: Synthetic peptide
ARDQRTGPFDY

SEQ ID NO: 159 - protein, 11 aa, Artificial Sequence
  Description of Artificial Sequence: Synthetic peptide
ARQAFAGPTDS

SEQ ID NO: 160 - protein, 15 aa, Artificial Sequence
  Description of Artificial Sequence: Synthetic peptide
ARRGPVNWNGSSLDV

SEQ ID NO: 161 - protein, 16 aa, Artificial Sequence
  Description of Artificial Sequence: Synthetic peptide
TRDRADSWNFHDYFDY

SEQ ID NO: 162 - protein, 11 aa, Artificial Sequence
  Description of Artificial Sequence: Synthetic peptide
AKIAVAGPVDY

SEQ ID NO: 163 - protein, 14 aa, Artificial Sequence
  Description of Artificial Sequence: Synthetic peptide
ATTYSGSDYYRLDV

SEQ ID NO: 164 - protein, 13 aa, Artificial Sequence
  Description of Artificial Sequence: Synthetic peptide
ARPDSLWGAAFDY

SEQ ID NO: 165 - protein, 11 aa, Artificial Sequence
  Description of Artificial Sequence: Synthetic peptide
ARIGAAGPGDY

SEQ ID NO: 166 - protein, 15 aa, Artificial Sequence
  Description of Artificial Sequence: Synthetic peptide
AKYWGDYYGYSSLDV

SEQ ID NO: 167 - protein, 11 aa, Artificial Sequence
  Description of Artificial Sequence: Synthetic peptide
ARVEVVGPTGY

SEQ ID NO: 168 - protein, 13 aa, Artificial Sequence
  Description of Artificial Sequence: Synthetic peptide
ARRYSGSYSPFDC

SEQ ID NO: 169 - protein, 18 aa, Artificial Sequence
  Description of Artificial Sequence: Synthetic peptide
AREGMGCTGSGCSISFDY

SEQ ID NO: 170 - protein, 13 aa, Artificial Sequence
  Description of Artificial Sequence: Synthetic peptide
ARQGYSGYSLFDY

SEQ ID NO: 171 - protein, 11 aa, Artificial Sequence
  Description of Artificial Sequence: Synthetic peptide
ASEIAGGPVDY

SEQ ID NO: 172 - protein, 15 aa, Artificial Sequence
  Description of Artificial Sequence: Synthetic peptide
ARDSSGWPWDNRFDV

SEQ ID NO: 173 - protein, 12 aa, Artificial Sequence
  Description of Artificial Sequence: Synthetic peptide
ARVTGRIAPFDY

SEQ ID NO: 174 - protein, 16 aa, Artificial Sequence
  Description of Artificial Sequence: Synthetic peptide
ATNIWTGYSFYYGLDS

SEQ ID NO: 175 - protein, 11 aa, Artificial Sequence
  Description of Artificial Sequence: Synthetic peptide
AREGRIHPLDS

SEQ ID NO: 176 - protein, 12 aa, Artificial Sequence
  Description of Artificial Sequence: Synthetic peptide
AKDHDYGGGLDS

SEQ ID NO: 177 - protein, 12 aa, Artificial Sequence
  Description of Artificial Sequence: Synthetic peptide
AKKSSGSWEVDY

SEQ ID NO: 178 - protein, 19 aa, Artificial Sequence
  Description of Artificial Sequence: Synthetic peptide
ARHAYYNIWTGYSTNRFDV

SEQ ID NO: 179 - protein, 13 aa, Artificial Sequence
  Description of Artificial Sequence: Synthetic peptide
AEGSGSWNGRFGV

SEQ ID NO: 180 - protein, 17 aa, Artificial Sequence
  Description of Artificial Sequence: Synthetic peptide
ATGRYYGGSYYGDRFDV

SEQ ID NO: 181 - protein, 12 aa, Artificial Sequence
  Description of Artificial Sequence: Synthetic peptide
AKCSSSSTGLDY

SEQ ID NO: 182 - protein, 18 aa, Artificial Sequence
  Description of Artificial Sequence: Synthetic peptide
ARDRSVTPFSWVEYYFDY

SEQ ID NO: 183 - protein, 11 aa, Artificial Sequence
  Description of Artificial Sequence: Synthetic peptide
VRVVKYGPLDY

SEQ ID NO: 184 - protein, 20 aa, Artificial Sequence
  Description of Artificial Sequence: Synthetic peptide
ARNPPYYNLWTGYYTHSLDV

SEQ ID NO: 185 - protein, 17 aa, Artificial Sequence
  Description of Artificial Sequence: Synthetic peptide
AREGYCSYTYCSNLFEF

SEQ ID NO: 186 - protein, 11 aa, Artificial Sequence
  Description of Artificial Sequence: Synthetic peptide
ARARIAAPFDY

SEQ ID NO: 187 - protein, 11 aa, Artificial Sequence
  Description of Artificial Sequence: Synthetic peptide
ARAGRMAATDY

SEQ ID NO: 188 - protein, 11 aa, Artificial Sequence
  Description of Artificial Sequence: Synthetic peptide
VRDVTLGPIDN

SEQ ID NO: 189 - protein, 11 aa, Artificial Sequence
  Description of Artificial Sequence: Synthetic peptide
AREGRIQPLDS

SEQ ID NO: 190 - protein, 11 aa, Artificial Sequence
  Description of Artificial Sequence: Synthetic peptide
AKCRNWNDFAY

SEQ ID NO: 191 - protein, 11 aa, Artificial Sequence
  Description of Artificial Sequence: Synthetic peptide
ARVHRGGPFDY

SEQ ID NO: 192 - protein, 11 aa, Artificial Sequence
  Description of Artificial Sequence: Synthetic peptide
ARGGRVHPMDY

SEQ ID NO: 193 - protein, 11 aa, Artificial Sequence
  Description of Artificial Sequence: Synthetic peptide
ARGGPVSPFDY

SEQ ID NO: 194 - protein, 11 aa, Artificial Sequence
  Description of Artificial Sequence: Synthetic peptide
ARGQRVAPFDV

SEQ ID NO: 195 - protein, 21 aa, Artificial Sequence
  Description of Artificial Sequence: Synthetic peptide
AKETYEDDYGYYSLGYNRFDV

SEQ ID NO: 196 - protein, 12 aa, Artificial Sequence
  Description of Artificial Sequence: Synthetic peptide
ASAWREHLPIDY

SEQ ID NO: 197 - protein, 16 aa, Artificial Sequence
  Description of Artificial Sequence: Synthetic peptide
ARDLYPGVINPSGLDS

SEQ ID NO: 198 - protein, 16 aa, Artificial Sequence
  Description of Artificial Sequence: Synthetic peptide
ARDKGSSYYQPEYFEF

SEQ ID NO: 199 - protein, 16 aa, Artificial Sequence
  Description of Artificial Sequence: Synthetic peptide
VRDKGSSYYQPEYFEF

SEQ ID NO: 200 - protein, 11 aa, Artificial Sequence
  Description of Artificial Sequence: Synthetic peptide
ARTGKAAPVDY

SEQ ID NO: 201 - protein, 11 aa, Artificial Sequence
  Description of Artificial Sequence: Synthetic peptide
ARTGKAAPVDC

SEQ ID NO: 202 - protein, 16 aa, Artificial Sequence
  Description of Artificial Sequence: Synthetic peptide
AKGGDNYYDSGYYDDY

SEQ ID NO: 203 - protein, 13 aa, Artificial Sequence
  Description of Artificial Sequence: Synthetic peptide
ARNRGWGDLVFDY

SEQ ID NO: 204 - protein, 14 aa, Artificial Sequence
  Description of Artificial Sequence: Synthetic peptide
AKVLSGWFWDYFDY

SEQ ID NO: 205 - protein, 11 aa, Artificial Sequence
  Description of Artificial Sequence: Synthetic peptide
ARLAVAGPVDY

SEQ ID NO: 206 - protein, 14 aa, Artificial Sequence
  Description of Artificial Sequence: Synthetic peptide
ARGSSGWYGSGLDS

SEQ ID NO: 207 - protein, 16 aa, Artificial Sequence
  Description of Artificial Sequence: Synthetic peptide
ARDHIESWNKVNWFDV

SEQ ID NO: 208 - protein, 14 aa, Artificial Sequence
  Description of Artificial Sequence: Synthetic peptide
ATYSGSWYAEYFEF

SEQ ID NO: 209 - protein, 17 aa, Artificial Sequence
  Description of Artificial Sequence: Synthetic peptide
AKQEDYNFWSSYFLPDY

SEQ ID NO: 210 - protein, 13 aa, Artificial Sequence
  Description of Artificial Sequence: Synthetic peptide
ARDSSGWYEGFDY

SEQ ID NO: 211 - protein, 15 aa, Artificial Sequence
  Description of Artificial Sequence: Synthetic peptide
ATGRYYGPSWAIFDY

SEQ ID NO: 212 - protein, 11 aa, Artificial Sequence
  Description of Artificial Sequence: Synthetic peptide
ARDGNFGPIDY

SEQ ID NO: 213 - protein, 9 aa, Artificial Sequence
  Description of Artificial Sequence: Synthetic peptide
ASGPNWFDV

SEQ ID NO: 214 - protein, 15 aa, Artificial Sequence
  Description of Artificial Sequence: Synthetic peptide
AKSETDFWTSYYFNY

SEQ ID NO: 215 - protein, 20 aa, Artificial Sequence
  Description of Artificial Sequence: Synthetic peptide
ARDICSGSGCYWYRDNWFDV

SEQ ID NO: 216 - protein, 11 aa, Artificial Sequence
  Description of Artificial Sequence: Synthetic peptide
ASNRRIAPLDY

SEQ ID NO: 217 - protein, 9 aa, Artificial Sequence
  Description of Artificial Sequence: Synthetic peptide
ASGRYYFDY

SEQ ID NO: 218 - protein, 15 aa, Artificial Sequence
  Description of Artificial Sequence: Synthetic peptide
ARDRTVTPNRGYFEF

SEQ ID NO: 219 - protein, 15 aa, Artificial Sequence
  Description of Artificial Sequence: Synthetic peptide
ARDGPYSGGWSELDS

SEQ ID NO: 220 - protein, 13 aa, Artificial Sequence
  Description of Artificial Sequence: Synthetic peptide
ARWEYSGNWGLDY

SEQ ID NO: 221 - protein, 16 aa, Artificial Sequence
  Description of Artificial Sequence: Synthetic peptide
ARSTSSWPRTSDAFDF

SEQ ID NO: 222 - protein, 12 aa, Artificial Sequence
  Description of Artificial Sequence: Synthetic peptide
AKKRSSWSRIDY

SEQ ID NO: 223 - protein, 14 aa, Artificial Sequence
  Description of Artificial Sequence: Synthetic peptide
ARDGSGWRRVTFDY

SEQ ID NO: 224 - protein, 9 aa, Artificial Sequence
  Description of Artificial Sequence: Synthetic peptide
ATGRNYFDY

SEQ ID NO: 225 - protein, 12 aa, Artificial Sequence
  Description of Artificial Sequence: Synthetic peptide
AKTGAVTTGFDY

SEQ ID NO: 226 - protein, 14 aa, Artificial Sequence
  Description of Artificial Sequence: Synthetic peptide
ARLVGGSGYYYIGD

SEQ ID NO: 227 - protein, 13 aa, Artificial Sequence
  Description of Artificial Sequence: Synthetic peptide
AKVPYSSWSHFDY

SEQ ID NO: 228 - protein, 14 aa, Artificial Sequence
  Description of Artificial Sequence: Synthetic peptide
TSPRMRYSSGSFDY

SEQ ID NO: 229 - protein, 14 aa, Artificial Sequence
  Description of Artificial Sequence: Synthetic peptide
ARVRGYSGYSFFDY

SEQ ID NO: 230 - protein, 13 aa, Artificial Sequence
  Description of Artificial Sequence: Synthetic peptide
SRGSTWSGDWFDV

SEQ ID NO: 231 - protein, 15 aa, Artificial Sequence
  Description of Artificial Sequence: Synthetic peptide
TKRLAYSNPYNRFDV

SEQ ID NO: 232 - protein, 27 aa, Artificial Sequence
  Description of Artificial Sequence: Synthetic peptide
ARGGVGLDDVTYYYSGSYYYHRTSFDY

SEQ ID NO: 233 - protein, 18 aa, Artificial Sequence
  Description of Artificial Sequence: Synthetic peptide
AGDRGGYNYGFTDNWFDV

SEQ ID NO: 234 - protein, 20 aa, Artificial Sequence
  Description of Artificial Sequence: Synthetic peptide
TRGTAYYNFWSNSSPGYFDY

SEQ ID NO: 235 - protein, 16 aa, Artificial Sequence
  Description of Artificial Sequence: Synthetic peptide
ARDKGSSYYQPESFEF

SEQ ID NO: 236 - protein, 27 aa, Artificial Sequence
  Description of Artificial Sequence: Synthetic peptide
ARRYYEDDYGYYYPGPNIAGTTRGVEE

SEQ ID NO: 237 - protein, 18 aa, Artificial Sequence
  Description of Artificial Sequence: Synthetic peptide
ARGITRMITVTKTNWFDV

SEQ ID NO: 238 - protein, 11 aa, Artificial Sequence
  Description of Artificial Sequence: Synthetic peptide
ARLAVAGPFDY

SEQ ID NO: 239 - protein, 11 aa, Artificial Sequence
  Description of Artificial Sequence: Synthetic peptide
ARLGVAGPLDY

SEQ ID NO: 240 - protein, 8 aa, Artificial Sequence
  Description of Artificial Sequence: Synthetic peptide
ATYKTIDY

SEQ ID NO: 241 - protein, 8 aa, Artificial Sequence
  Description of Artificial Sequence: Synthetic peptide
ASYKNIDY

SEQ ID NO: 242 - protein, 11 aa, Artificial Sequence
  Description of Artificial Sequence: Synthetic peptide
ARDRHGIPFDY

SEQ ID NO: 243 - protein, 13 aa, Artificial Sequence
  Description of Artificial Sequence: Synthetic peptide
ARSRGYWGDLFDF

SEQ ID NO: 244 - protein, 13 aa, Artificial Sequence
  Description of Artificial Sequence: Synthetic peptide
ARLSGWGDFRIDY

SEQ ID NO: 245 - protein, 8 aa, Artificial Sequence
  Description of Artificial Sequence: Synthetic peptide
ATGIWFDV

SEQ ID NO: 246 - protein, 11 aa, Artificial Sequence
  Description of Artificial Sequence: Synthetic peptide
ARANNGGYFDY

SEQ ID NO: 247 - protein, 15 aa, Artificial Sequence
  Description of Artificial Sequence: Synthetic peptide
ARMTTVAAFGGYFDL

SEQ ID NO: 248 - protein, 9 aa, Artificial Sequence
  Description of Artificial Sequence: Synthetic peptide
ASGGNYADY

SEQ ID NO: 249 - protein, 11 aa, Artificial Sequence
  Description of Artificial Sequence: Synthetic peptide
ARRLSRRYFDY

SEQ ID NO: 250 - protein, 16 aa, Artificial Sequence
  Description of Artificial Sequence: Synthetic peptide
TREFCSGIYCYAPFDY

SEQ ID NO: 251 - protein, 8 aa, Artificial Sequence
  Description of Artificial Sequence: Synthetic peptide
ASFKTLDV

SEQ ID NO: 252 - protein, 14 aa, Artificial Sequence
  Description of Artificial Sequence: Synthetic peptide
AKGVGGFSYSYPHY

SEQ ID NO: 253 - protein, 14 aa, Artificial Sequence
  Description of Artificial Sequence: Synthetic peptide
ARDGHYNFWSPPGY

SEQ ID NO: 254 - protein, 14 aa, Artificial Sequence
  Description of Artificial Sequence: Synthetic peptide
ARAEDEDDYGSFDV

SEQ ID NO: 255 - protein, 16 aa, Artificial Sequence
  Description of Artificial Sequence: Synthetic peptide
ARLGSSGWYRDDAFDF

SEQ ID NO: 256 - protein, 11 aa, Artificial Sequence
  Description of Artificial Sequence: Synthetic peptide
AKPRGRWLEDY

SEQ ID NO: 257 - protein, 11 aa, Artificial Sequence
  Description of Artificial Sequence: Synthetic peptide
TRPRQYSTGDY

SEQ ID NO: 258 - protein, 17 aa, Artificial Sequence
  Description of Artificial Sequence: Synthetic peptide
AKMGGRGYSSYGPVFDY

SEQ ID NO: 259 - protein, 11 aa, Artificial Sequence
  Description of Artificial Sequence: Synthetic peptide
ARIVTRGPFDY

SEQ ID NO: 260 - protein, 17 aa, Artificial Sequence
  Description of Artificial Sequence: Synthetic peptide
ARDVTTRVVIIDHRFDV

SEQ ID NO: 261 - protein, 14 aa, Artificial Sequence
  Description of Artificial Sequence: Synthetic peptide
ARQLGGGQTDRFDV

SEQ ID NO: 262 - protein, 11 aa, Artificial Sequence
  Description of Artificial Sequence: Synthetic peptide
ARQAYSNYPDY

SEQ ID NO: 263 - protein, 12 aa, Artificial Sequence
  Description of Artificial Sequence: Synthetic peptide
VKLREKWETRGD

SEQ ID NO: 264 - protein, 13 aa, Artificial Sequence
  Description of Artificial Sequence: Synthetic peptide
AKSYGSMSNRFDV

SEQ ID NO: 265 - protein, 11 aa, Artificial Sequence
  Description of Artificial Sequence: Synthetic peptide
ARVIRLGPFDY

SEQ ID NO: 266 - protein, 22 aa, Artificial Sequence
  Description of Artificial Sequence: Synthetic peptide
ARETFEGDDYGYYYTPDNWFDV

SEQ ID NO: 267 - protein, 14 aa, Artificial Sequence
  Description of Artificial Sequence: Synthetic peptide
AKSGNSGSWNYFDY

SEQ ID NO: 268 - protein, 13 aa, Artificial Sequence
  Description of Artificial Sequence: Synthetic peptide
ARRRGWGDPYFDY

SEQ ID NO: 269 - protein, 14 aa, Artificial Sequence
  Description of Artificial Sequence: Synthetic peptide
ATGFSMITVALFDF

SEQ ID NO: 270 - protein, 18 aa, Artificial Sequence
  Description of Artificial Sequence: Synthetic peptide
ASQGYEDDYAYWAFKFDY

SEQ ID NO: 271 - protein, 12 aa, Artificial Sequence
  Description of Artificial Sequence: Synthetic peptide
ARSPGIVAPFDY

SEQ ID NO: 272 - protein, 15 aa, Artificial Sequence
  Description of Artificial Sequence: Synthetic peptide
ARSRSGSNSESRFDV

SEQ ID NO: 273 - protein, 17 aa, Artificial Sequence
  Description of Artificial Sequence: Synthetic peptide
ARPLYSGNWNVYWYFDL

SEQ ID NO: 274 - protein, 12 aa, Artificial Sequence
  Description of Artificial Sequence: Synthetic peptide
ARDGWGGWTIDY

SEQ ID NO: 275 - protein, 13 aa, Artificial Sequence
  Description of Artificial Sequence: Synthetic peptide
ARSGYGSGGTFDY

SEQ ID NO: 276 - protein, 16 aa, Artificial Sequence
  Description of Artificial Sequence: Synthetic peptide
ATTPGYCSSTYCRFDY

SEQ ID NO: 277 - protein, 19 aa, Artificial Sequence
  Description of Artificial Sequence: Synthetic peptide
ATKNYYDSGYHLSGEYFEF

SEQ ID NO: 278 - protein, 15 aa, Artificial Sequence
  Description of Artificial Sequence: Synthetic peptide
AQCPEYSWNMGWFDV

SEQ ID NO: 279 - protein, 16 aa, Artificial Sequence
  Description of Artificial Sequence: Synthetic peptide
ASPFYGSGYYTRRFDV

SEQ ID NO: 280 - protein, 18 aa, Artificial Sequence
  Description of Artificial Sequence: Synthetic peptide
ARDGYYSGDYYRHNWFAV

SEQ ID NO: 281 - protein, 10 aa, Artificial Sequence
  Description of Artificial Sequence: Synthetic peptide
ARDCVDAFDY

SEQ ID NO: 282 - protein, 12 aa, Artificial Sequence
  Description of Artificial Sequence: Synthetic peptide
ATGYNWNDPFDY

SEQ ID NO: 283 - protein, 16 aa, Artificial Sequence
  Description of Artificial Sequence: Synthetic peptide
TKVEGGYWGDYHRFDV

SEQ ID NO: 284 - protein, 11 aa, Artificial Sequence
  Description of Artificial Sequence: Synthetic peptide
QSYDSSLSGHL

SEQ ID NO: 285 - protein, 11 aa, Artificial Sequence
  Description of Artificial Sequence: Synthetic peptide
QSYDSSLSAGL

SEQ ID NO: 286 - protein, 11 aa, Artificial Sequence
  Description of Artificial Sequence: Synthetic peptide
QSYDSSLSAHV

SEQ ID NO: 287 - protein, 11 aa, Artificial Sequence
  Description of Artificial Sequence: Synthetic peptide
QSYDNSLSAWV

SEQ ID NO: 288 - protein, 11 aa, Artificial Sequence
  Description of Artificial Sequence: Synthetic peptide
QSYDSSLSVRV

SEQ ID NO: 289 - protein, 11 aa, Artificial Sequence
  Description of Artificial Sequence: Synthetic peptide
QSYDNSLSARV

SEQ ID NO: 290 - protein, 11 aa, Artificial Sequence
  Description of Artificial Sequence: Synthetic peptide
  MOD_RES (9)..(9): Any amino acid
QSYDNSLSXQV

SEQ ID NO: 291 - protein, 11 aa, Artificial Sequence
  Description of Artificial Sequence: Synthetic peptide
QSYDNSLSAHV

SEQ ID NO: 292 - protein, 11 aa, Artificial Sequence
  Description of Artificial Sequence: Synthetic peptide
QSYDSSLSADV

SEQ ID NO: 293 - protein, 11 aa, Artificial Sequence
  Description of Artificial Sequence: Synthetic peptide
LSYDSSLSAHI

SEQ ID NO: 294 - protein, 11 aa, Artificial Sequence
  Description of Artificial Sequence: Synthetic peptide
QVWDSSSDHPL

SEQ ID NO: 295 - protein, 11 aa, Artificial Sequence
  Description of Artificial Sequence: Synthetic peptide
GAWDSSLSAGL

SEQ ID NO: 296 - protein, 11 aa, Artificial Sequence
  Description of Artificial Sequence: Synthetic peptide
SAWDSSLSDVL

SEQ ID NO: 297 - protein, 11 aa, Artificial Sequence
  Description of Artificial Sequence: Synthetic peptide
AAWDDSLSGVL

SEQ ID NO: 298 - protein, 11 aa, Artificial Sequence
  Description of Artificial Sequence: Synthetic peptide
ETWDYSLNGPL

SEQ ID NO: 299 - protein, 9 aa, Artificial Sequence
  Description of Artificial Sequence: Synthetic peptide
YSGDDNNDV

SEQ ID NO: 300 - protein, 11 aa, Artificial Sequence
  Description of Artificial Sequence: Synthetic peptide
QSYDSSLSGHI

SEQ ID NO: 301 - protein, 7 aa, Artificial Sequence
  Description of Artificial Sequence: Synthetic peptide
QTWTTDV

SEQ ID NO: 302 - protein, 10 aa, Artificial Sequence
  Description of Artificial Sequence: Synthetic peptide
CSYTTSNTLL

SEQ ID NO: 303 - protein, 12 aa, Artificial Sequence
  Description of Artificial Sequence: Synthetic peptide
QSYDSSLSVHYI

SEQ ID NO: 304 - protein, 10 aa, Artificial Sequence
  Description of Artificial Sequence: Synthetic peptide
SSYASSSTWV

SEQ ID NO: 305 - protein, 11 aa, Artificial Sequence
  Description of Artificial Sequence: Synthetic peptide
QSYDSSLSAVL

SEQ ID NO: 306 - protein, 11 aa, Artificial Sequence
  Description of Artificial Sequence: Synthetic peptide
QSYDSSLSALL

SEQ ID NO: 307 - protein, 11 aa, Artificial Sequence
  Description of Artificial Sequence: Synthetic peptide
QSYDSSLSAVF

SEQ ID NO: 308 - protein, 11 aa, Artificial Sequence
  Description of Artificial Sequence: Synthetic peptide
QSYDSSLSARL

SEQ ID NO: 309 - protein, 11 aa, Artificial Sequence
  Description of Artificial Sequence: Synthetic peptide
QSYDSSLSNVL

SEQ ID NO: 310 - protein, 11 aa, Artificial Sequence
  Description of Artificial Sequence: Synthetic peptide
QSYDSSLSGVL

SEQ ID NO: 311 - protein, 11 aa, Artificial Sequence
  Description of Artificial Sequence: Synthetic peptide
QSYDNSLSAVL

SEQ ID NO: 312 - protein, 11 aa, Artificial Sequence
  Description of Artificial Sequence: Synthetic peptide
QSYDNNLSAVL

SEQ ID NO: 313 - protein, 11 aa, Artificial Sequence
  Description of Artificial Sequence: Synthetic peptide
QSYDSSLSAQV

SEQ ID NO: 314 - protein, 11 aa, Artificial Sequence
  Description of Artificial Sequence: Synthetic peptide
QSYDSSLSAHL

SEQ ID NO: 315 - protein, 11 aa, Artificial Sequence
  Description of Artificial Sequence: Synthetic peptide
QSYDSSLSAWV

SEQ ID NO: 316 - protein, 11 aa, Artificial Sequence
  Description of Artificial Sequence: Synthetic peptide
QSYDSYLSAGL

SEQ ID NO: 317 - protein, 11 aa, Artificial Sequence
  Description of Artificial Sequence: Synthetic peptide
QSYDNSLSDDV

SEQ ID NO: 318 - protein, 11 aa, Artificial Sequence
  Description of Artificial Sequence: Synthetic peptide
QSYDSSLSALV

SEQ ID NO: 319 - protein, 12 aa, Artificial Sequence
  Description of Artificial Sequence: Synthetic peptide
QSYDSNLSAHVL

SEQ ID NO: 320 - protein, 12 aa, Artificial Sequence
  Description of Artificial Sequence: Synthetic peptide
QSFDSNLSIHLL

SEQ ID NO: 321 - protein, 12 aa, Artificial Sequence
  Description of Artificial Sequence: Synthetic peptide
QSYDSSLSAHVL

SEQ ID NO: 322 - protein, 11 aa, Artificial Sequence
  Description of Artificial Sequence: Synthetic peptide
QSYDSSLSAYI

SEQ ID NO: 323 - protein, 11 aa, Artificial Sequence
  Description of Artificial Sequence: Synthetic peptide
DSWDSGGTHVL

SEQ ID NO: 324 - protein, 11 aa, Artificial Sequence
  Description of Artificial Sequence: Synthetic peptide
AAWDDSLSGPV

SEQ ID NO: 325 - protein, 11 aa, Artificial Sequence
  Description of Artificial Sequence: Synthetic peptide
QVWDSRSDHPL

SEQ ID NO: 326 - protein, 9 aa, Artificial Sequence
  Description of Artificial Sequence: Synthetic peptide
MIWHNNASI

SEQ ID NO: 327 - protein, 10 aa, Artificial Sequence
  Description of Artificial Sequence: Synthetic peptide
WLYYSGGHGL

SEQ ID NO: 328 - protein, 12 aa, Artificial Sequence
  Description of Artificial Sequence: Synthetic peptide
QVWDSSSDHHDV

SEQ ID NO: 329 - protein, 11 aa, Artificial Sequence
  Description of Artificial Sequence: Synthetic peptide
QSYDSSLRAQV

SEQ ID NO: 330 - protein, 11 aa, Artificial Sequence
  Description of Artificial Sequence: Synthetic peptide
QSHDSSLTAGL

SEQ ID NO: 331 - protein, 11 aa, Artificial Sequence
  Description of Artificial Sequence: Synthetic peptide
QSHDSSLSAGL

SEQ ID NO: 332 - protein, 11 aa, Artificial Sequence
  Description of Artificial Sequence: Synthetic peptide
AAWDDSLKGWV

SEQ ID NO: 333 - protein, 11 aa, Artificial Sequence
  Description of Artificial Sequence: Synthetic peptide
AAWDDSLSGWV

SEQ ID NO: 334 - protein, 11 aa, Artificial Sequence
  Description of Artificial Sequence: Synthetic peptide
AAWDDSLNGWV

SEQ ID NO: 335 - protein, 11 aa, Artificial Sequence
  Description of Artificial Sequence: Synthetic peptide
AAWDDSLSGPL

SEQ ID NO: 336 - protein, 9 aa, Artificial Sequence
  Description of Artificial Sequence: Synthetic peptide
MIWHNNVWA

SEQ ID NO: 337 - protein, 9 aa, Artificial Sequence
  Description of Artificial Sequence: Synthetic peptide
VIWHNNVWA

SEQ ID NO: 338 - protein, 9 aa, Artificial Sequence
  Description of Artificial Sequence: Synthetic peptide
MIWHNNAWI

SEQ ID NO: 339 - protein, 9 aa, Artificial Sequence
  Description of Artificial Sequence: Synthetic peptide
MIWHNNAWV

SEQ ID NO: 340 - protein, 11 aa, Artificial Sequence
  Description of Artificial Sequence: Synthetic peptide
AAWDDSLSGYI

SEQ ID NO: 341 - protein, 11 aa, Artificial Sequence
  Description of Artificial Sequence: Synthetic peptide
QSYDNSLSAYI

SEQ ID NO: 342 - protein, 11 aa, Artificial Sequence
  Description of Artificial Sequence: Synthetic peptide
QSYDSILSSYI

SEQ ID NO: 343 - protein, 11 aa, Artificial Sequence
  Description of Artificial Sequence: Synthetic peptide
QSYDSRLSADV

SEQ ID NO: 344 - protein, 12 aa, Artificial Sequence
  Description of Artificial Sequence: Synthetic peptide
QVWDGSTKYAGL

SEQ ID NO: 345 - protein, 12 aa, Artificial Sequence
  Description of Artificial Sequence: Synthetic peptide
QVWDDSTNYAGL

SEQ ID NO: 346 - protein, 11 aa, Artificial Sequence
  Description of Artificial Sequence: Synthetic peptide
GAWDSSLSALL

SEQ ID NO: 347 - protein, 11 aa, Artificial Sequence
  Description of Artificial Sequence: Synthetic peptide
QSYDSSLSDVL

SEQ ID NO: 348 - protein, 11 aa, Artificial Sequence
  Description of Artificial Sequence: Synthetic peptide
QSYDSSLSAQL

SEQ ID NO: 349 - protein, 10 aa, Artificial Sequence
  Description of Artificial Sequence: Synthetic peptide
MIWHEDDFVL

SEQ ID NO: 350 - protein, 12 aa, Artificial Sequence
  Description of Artificial Sequence: Synthetic peptide
GAWDSSLSAHWV

SEQ ID NO: 351 - protein, 11 aa, Artificial Sequence
  Description of Artificial Sequence: Synthetic peptide
DSWDSSGTHVL

SEQ ID NO: 352 - protein, 10 aa, Artificial Sequence
  Description of Artificial Sequence: Synthetic peptide
SSYVGSGTYI

SEQ ID NO: 353 - protein, 10 aa, Artificial Sequence
  Description of Artificial Sequence: Synthetic peptide
SSYAGSGTGL

SEQ ID NO: 354 - protein, 10 aa, Artificial Sequence
  Description of Artificial Sequence: Synthetic peptide
CSYTTSNTLI

SEQ ID NO: 355 - protein, 11 aa, Artificial Sequence
  Description of Artificial Sequence: Synthetic peptide
QVWDISSDHPV

SEQ ID NO: 356 - protein, 11 aa, Artificial Sequence
  Description of Artificial Sequence: Synthetic peptide
QVWDSSSAHPV

SEQ ID NO: 357 - protein, 12 aa, Artificial Sequence
  Description of Artificial Sequence: Synthetic peptide
QSYDSSLSAHYI

SEQ ID NO: 358 - protein, 11 aa, Artificial Sequence
  Description of Artificial Sequence: Synthetic peptide
QSADSSGNHWV

SEQ ID NO: 359 - protein, 9 aa, Artificial Sequence
  Description of Artificial Sequence: Synthetic peptide
QTWTTGIHV

SEQ ID NO: 360 - protein, 10 aa, Artificial Sequence
  Description of Artificial Sequence: Synthetic peptide
GSYRTGATFL

SEQ ID NO: 361 - protein, 10 aa, Artificial Sequence
  Description of Artificial Sequence: Synthetic peptide
SSYAGSNTFI

SEQ ID NO: 362 - protein, 11 aa, Artificial Sequence
  Description of Artificial Sequence: Synthetic peptide
QVWDSSSDHWV

SEQ ID NO: 363 - protein, 11 aa, Artificial Sequence
  Description of Artificial Sequence: Synthetic peptide
QSYDGSLSAQL

SEQ ID NO: 364 - protein, 9 aa, Artificial Sequence
  Description of Artificial Sequence: Synthetic peptide
QVWDSDHPL

SEQ ID NO: 365 - protein, 11 aa, Artificial Sequence
  Description of Artificial Sequence: Synthetic peptide
QSYDSTLSGGL

SEQ ID NO: 366 - protein, 11 aa, Artificial Sequence
  Description of Artificial Sequence: Synthetic peptide
QSYDSSLSGGL

SEQ ID NO: 367 - protein, 11 aa, Artificial Sequence
  Description of Artificial Sequence: Synthetic peptide
QSYDNTLSAGL

SEQ ID NO: 368 - protein, 11 aa, Artificial Sequence
  Description of Artificial Sequence: Synthetic peptide
QSYDSSLSVGL

SEQ ID NO: 369 - protein, 11 aa, Artificial Sequence
  Description of Artificial Sequence: Synthetic peptide
QSYDSSLTAGL

SEQ ID NO: 370 - protein, 11 aa, Artificial Sequence
  Description of Artificial Sequence: Synthetic peptide
QSYDNNLSAQV

SEQ ID NO: 371 - protein, 11 aa, Artificial Sequence
  Description of Artificial Sequence: Synthetic peptide
QSYDSSLSARV

SEQ ID NO: 372 - protein, 11 aa, Artificial Sequence
  Description of Artificial Sequence: Synthetic peptide
QSYDISLSAGL

SEQ ID NO: 373 - protein, 11 aa, Artificial Sequence
  Description of Artificial Sequence: Synthetic peptide
QSYDNILNAGL

SEQ ID NO: 374 - protein, 11 aa, Artificial Sequence
  Description of Artificial Sequence: Synthetic peptide
HSYDSSLSAQV

SEQ ID NO: 375 - protein, 11 aa, Artificial Sequence
  Description of Artificial Sequence: Synthetic peptide
QSYDNSLSAVI

SEQ ID NO: 376 - protein, 11 aa, Artificial Sequence
  Description of Artificial Sequence: Synthetic peptide
  MOD_RES (9)..(9): Any amino acid
QSYDSSLSXVL

SEQ ID NO: 377 - protein, 11 aa, Artificial Sequence
  Description of Artificial Sequence: Synthetic peptide
QSYDSRLSALL

SEQ ID NO: 378 - protein, 11 aa, Artificial Sequence
  Description of Artificial Sequence: Synthetic peptide
QSYDSSLSAVV

SEQ ID NO: 379 - protein, 11 aa, Artificial Sequence
  Description of Artificial Sequence: Synthetic peptide
QSYDNSLSALL

SEQ ID NO: 380 - protein, 11 aa, Artificial Sequence
  Description of Artificial Sequence: Synthetic peptide
  MOD_RES (7)..(9): Any amino acid
QSYDSSXXXHV

SEQ ID NO: 381 - protein, 11 aa, Artificial Sequence
  Description of Artificial Sequence: Synthetic peptide
QSYDSSLSTHV

SEQ ID NO: 382 - protein, 11 aa, Artificial Sequence
  Description of Artificial Sequence: Synthetic peptide
QSYDSSLTADV

SEQ ID NO: 383 - protein, 10 aa, Artificial Sequence
  Description of Artificial Sequence: Synthetic peptide
SSYAGSNTYI

SEQ ID NO: 384 - protein, 10 aa, Artificial Sequence
  Description of Artificial Sequence: Synthetic peptide
SSYAGSGTYI

SEQ ID NO: 385 - protein, 11 aa, Artificial Sequence
  Description of Artificial Sequence: Synthetic peptide
QSYDSRLSAHV

SEQ ID NO: 386 - protein, 11 aa, Artificial Sequence
  Description of Artificial Sequence: Synthetic peptide
QSYHSSLRAYI

SEQ ID NO: 387 - protein, 10 aa, Artificial Sequence
  Description of Artificial Sequence: Synthetic peptide
RSYRSGRTNI

SEQ ID NO: 388 - protein, 10 aa, Artificial Sequence
  Description of Artificial Sequence: Synthetic peptide
CSYRSGDTLI

SEQ ID NO: 389 - protein, 10 aa, Artificial Sequence
  Description of Artificial Sequence: Synthetic peptide
YSYRSGNTLV

SEQ ID NO: 390 - protein, 10 aa, Artificial Sequence
  Description of Artificial Sequence: Synthetic peptide
CSYRSGSTFL

SEQ ID NO: 391 - protein, 10 aa, Artificial Sequence
  Description of Artificial Sequence: Synthetic peptide
CSYTTSSTFI

SEQ ID NO: 392 - protein, 10 aa, Artificial Sequence
  Description of Artificial Sequence: Synthetic peptide
SSYAGINTLV

SEQ ID NO: 393 - protein, 10 aa, Artificial Sequence
  Description of Artificial Sequence: Synthetic peptide
SSYAGSNTFL

SEQ ID NO: 394 - protein, 11 aa, Artificial Sequence
  Description of Artificial Sequence: Synthetic peptide
QVWDSSSDHPV

SEQ ID NO: 395 - protein, 11 aa, Artificial Sequence
  Description of Artificial Sequence: Synthetic peptide
QVWDSSNDHYI

SEQ ID NO: 396 - protein, 11 aa, Artificial Sequence
  Description of Artificial Sequence: Synthetic peptide
AAWDDRLSGWV

SEQ ID NO: 397 - protein, 10 aa, Artificial Sequence
  Description of Artificial Sequence: Synthetic peptide
CSYTSGSTWV

SEQ ID NO: 398 - protein, 10 aa, Artificial Sequence
  Description of Artificial Sequence: Synthetic peptide
DSWDSSGTLV

SEQ ID NO: 399 - protein, 11 aa, Artificial Sequence
  Description of Artificial Sequence: Synthetic peptide
LSYDSSLSAGL

SEQ ID NO: 400 - protein, 11 aa, Artificial Sequence
  Description of Artificial Sequence: Synthetic peptide
QVWDSSSDHVL

SEQ ID NO: 401 - protein, 11 aa, Artificial Sequence
  Description of Artificial Sequence: Synthetic peptide
QVWDNSSDHYI

SEQ ID NO: 402 - protein, 8 aa, Artificial Sequence
  Description of Artificial Sequence: Synthetic peptide
QVWDSSCK

SEQ ID NO: 403 - protein, 11 aa, Artificial Sequence
  Description of Artificial Sequence: Synthetic peptide
SAWDSSLSAYI

SEQ ID NO: 404 - protein, 12 aa, Artificial Sequence
  Description of Artificial Sequence: Synthetic peptide
QSYDSRLRVNWV

SEQ ID NO: 405 - protein, 11 aa, Artificial Sequence
  Description of Artificial Sequence: Synthetic peptide
EAWDRSLSAWV

SEQ ID NO: 406 - protein, 11 aa, Artificial Sequence
  Description of Artificial Sequence: Synthetic peptide
DTWDNSLNGYI

SEQ ID NO: 407 - protein, 16 aa, Artificial Sequence
  Description of Artificial Sequence: Synthetic peptide
ARLGEYSWNSIGYFDY

SEQ ID NO: 408 - protein, 14 aa, Artificial Sequence
  Description of Artificial Sequence: Synthetic peptide
ARGGYYSGRVFDDY

SEQ ID NO: 409 - protein, 13 aa, Artificial Sequence
  Description of Artificial Sequence: Synthetic peptide
ARHSGWGDPYLDV

SEQ ID NO: 410 - protein, 13 aa, Artificial Sequence
  Description of Artificial Sequence: Synthetic peptide
AINSGSWNYYFDY

SEQ ID NO: 411 - protein, 15 aa, Artificial Sequence
  Description of Artificial Sequence: Synthetic peptide
TSDPATYSWNEYFEF

SEQ ID NO: 412 - protein, 14 aa, Artificial Sequence
  Description of Artificial Sequence: Synthetic peptide
AKEDGGWSNNRVDV

SEQ ID NO: 413 - protein, 11 aa, Artificial Sequence
  Description of Artificial Sequence: Synthetic peptide
AKGRGYNRFDV

SEQ ID NO: 414 - protein, 14 aa, Artificial Sequence
  Description of Artificial Sequence: Synthetic peptide
VRQGYSSWYNSLDV

SEQ ID NO: 415 - protein, 19 aa, Artificial Sequence
  Description of Artificial Sequence: Synthetic peptide
ARDMRDIAAGGYTYGYFDY

SEQ ID NO: 416 - protein, 17 aa, Artificial Sequence
  Description of Artificial Sequence: Synthetic peptide
VRDPSITPGPSYNRFDV

SEQ ID NO: 417 - protein, 13 aa, Artificial Sequence
  Description of Artificial Sequence: Synthetic peptide
AKGVYGSTNRFDV

SEQ ID NO: 418 - protein, 13 aa, Artificial Sequence
  Description of Artificial Sequence: Synthetic peptide
AKGVYGLTNRFDV

SEQ ID NO: 419 - protein, 20 aa, Artificial Sequence
  Description of Artificial Sequence: Synthetic peptide
TKEGGPEYYNIWTGWNRFDV

SEQ ID NO: 420 - protein, 16 aa, Artificial Sequence
  Description of Artificial Sequence: Synthetic peptide
AGGYLLFPLGYNSLDV

SEQ ID NO: 421 - protein, 15 aa, Artificial Sequence
  Description of Artificial Sequence: Synthetic peptide
AKGGGPPSWNDPFDF

SEQ ID NO: 422 - protein, 13 aa, Artificial Sequence
  Description of Artificial Sequence: Synthetic peptide
AKNGPPYWGMGDY

SEQ ID NO: 423 - protein, 16 aa, Artificial Sequence
  Description of Artificial Sequence: Synthetic peptide
AKDRGRGGSWSLGNDY

SEQ ID NO: 424 - protein, 17 aa, Artificial Sequence
  Description of Artificial Sequence: Synthetic peptide
AKGGEDDYIYYYTGADY

SEQ ID NO: 425 - protein, 19 aa, Artificial Sequence
  Description of Artificial Sequence: Synthetic peptide
ARGLFNFWSGYWGHNSLDV

SEQ ID NO: 426 - protein, 15 aa, Artificial Sequence
  Description of Artificial Sequence: Synthetic peptide
ARDYSSWPTYNSLDV

SEQ ID NO: 427 - protein, 12 aa, Artificial Sequence
  Description of Artificial Sequence: Synthetic peptide
AKSTLLRRSLDY

SEQ ID NO: 428 - protein, 18 aa, Artificial Sequence
  Description of Artificial Sequence: Synthetic peptide
AKDGGPSGSYYYGGRFDV

SEQ ID NO: 429 - protein, 18 aa, Artificial Sequence
  Description of Artificial Sequence: Synthetic peptide
AKDGGPSGSYYYRGRFDV

SEQ ID NO: 430 - protein, 11 aa, Artificial Sequence
  Description of Artificial Sequence: Synthetic peptide
ARGGGHSSFDF

SEQ ID NO: 431 - protein, 13 aa, Artificial Sequence
  Description of Artificial Sequence: Synthetic peptide
ARDSYKDSPAFDF

SEQ ID NO: 432 - protein, 17 aa, Artificial Sequence
  Description of Artificial Sequence: Synthetic peptide
AKDQTDLDWLLYGGFDY

SEQ ID NO: 433 - protein, 11 aa, Artificial Sequence
  Description of Artificial Sequence: Synthetic peptide
QSYDNSLSAQV

SEQ ID NO: 434 - protein, 12 aa, Artificial Sequence
  Description of Artificial Sequence: Synthetic peptide
HIWDSRVPTKWV

SEQ ID NO: 435 - protein, 12 aa, Artificial Sequence
  Description of Artificial Sequence: Synthetic peptide
HIWDSRRPTNWV

SEQ ID NO: 436 - protein, 12 aa, Artificial Sequence
  Description of Artificial Sequence: Synthetic peptide
HIYDARGGTNWV

SEQ ID NO: 437 - protein, 12 aa, Artificial Sequence
  Description of Artificial Sequence: Synthetic peptide
HMWDSRSGFSWS

SEQ ID NO: 438 - protein, 11 aa, Artificial Sequence
  Description of Artificial Sequence: Synthetic peptide
MWDSRSGFSWS

SEQ ID NO: 439 - protein, 11 aa, Artificial Sequence
  Description of Artificial Sequence: Synthetic peptide
QSSDTSDSYKM

SEQ ID NO: 440 - protein, 10 aa, Artificial Sequence
  Description of Artificial Sequence: Synthetic peptide
GSLVGNWDVI

SEQ ID NO: 441 - protein, 10 aa, Artificial Sequence
  Description of Artificial Sequence: Synthetic peptide
SSLVGNWDVI

SEQ ID NO: 442 - protein, 10 aa, Artificial Sequence
  Description of Artificial Sequence: Synthetic peptide
SSLFGRWDVV

SEQ ID NO: 443 - protein, 10 aa, Artificial Sequence
  Description of Artificial Sequence: Synthetic peptide
SSLSGRWDIV

SEQ ID NO: 444 - protein, 9 aa, Artificial Sequence
  Description of Artificial Sequence: Synthetic peptide
SFGGSATVV

SEQ ID NO: 445 - protein, 12 aa, Artificial Sequence
  Description of Artificial Sequence: Synthetic peptide
QVWDSSSDHPWV

SEQ ID NO: 446 - protein, 10 aa, Artificial Sequence
  Description of Artificial Sequence: Synthetic peptide
  MOD_RES (8)..(10): Any amino acid
SSYAGSNXXX

SEQ ID NO: 447 - protein, 9 aa, Artificial Sequence
  Description of Artificial Sequence: Synthetic peptide
SYAGSSTVI

SEQ ID NO: 448 - DNA, 24 bp, Artificial Sequence
  Description of Artificial Sequence: Synthetic primer
acaggtgcccactcccaggtgcag

SEQ ID NO: 449 - DNA, 23 bp, Artificial Sequence
  Description of Artificial Sequence: Synthetic primer
aaggtgtccagtgtgargtgcag

SEQ ID NO: 450 - DNA, 27 bp, Artificial Sequence
  Description of Artificial Sequence: Synthetic primer
cccagatgggtcctgtcccaggtgcag

SEQ ID NO: 451 - DNA, 24 bp, Artificial Sequence
  Description of Artificial Sequence: Synthetic primer
caaggagtctgttccgaggtgcag

SEQ ID NO: 452 - DNA, 17 bp, Artificial Sequence
  Description of Artificial Sequence: Synthetic primer
ttctccaaggagtctgt

SEQ ID NO: 453 - DNA, 17 bp, Artificial Sequence
  Description of Artificial Sequence: Synthetic primer
taaaaggtgtccagtgt

SEQ ID NO: 454 - DNA, 17 bp, Artificial Sequence
  Description of Artificial Sequence: Synthetic primer
taagaggtgtccagtgt

SEQ ID NO: 455 - DNA, 17 bp, Artificial Sequence
  Description of Artificial Sequence: Synthetic primer
tagaaggtgtccagtgt

SEQ ID NO: 456 - DNA, 20 bp, Artificial Sequence
  Description of Artificial Sequence: Synthetic primer
atgaaacatctgtggttctt

SEQ ID NO: 457 - DNA, 17 bp, Artificial Sequence
  Description of Artificial Sequence: Synthetic primer
tacaaggtgtccagtgt

SEQ ID NO: 458 - DNA, 17 bp, Artificial Sequence
  Description of Artificial Sequence: Synthetic primer
ttaaagctgtccagtgt

SEQ ID NO: 459 - DNA, 20 bp, Artificial Sequence
  Description of Artificial Sequence: Synthetic primer
gctgaggagacggtgaccag

SEQ ID NO: 460 - DNA, 21 bp, Artificial Sequence
  Description of Artificial Sequence: Synthetic primer
gctgaggagatggtgattggg

SEQ ID NO: 461 - DNA, 21 bp, Artificial Sequence
  Description of Artificial Sequence: Synthetic primer
gctgaagagacggtgaccctg

SEQ ID NO: 462 - DNA, 21 bp, Artificial Sequence
  Description of Artificial Sequence: Synthetic primer
gctgaggagacggtgacgacg

SEQ ID NO: 463 - DNA, 48 bp, Artificial Sequence
  Description of Artificial Sequence: Synthetic primer
ctagtagcaactgcaaccggtgtacattcccaggtgcagctggtgcag

SEQ ID NO: 464 - DNA, 48 bp, Artificial Sequence
  Description of Artificial Sequence: Synthetic primer
ctagtagcaactgcaaccggtgtacattccgaggtgcagctggtgcag

SEQ ID NO: 465 - DNA, 48 bp, Artificial Sequence
  Description of Artificial Sequence: Synthetic primer
ctagtagcaactgcaaccggtgtacattcccaggttcagctggtgcag

SEQ ID NO: 466 - DNA, 48 bp, Artificial Sequence
  Description of Artificial Sequence: Synthetic primer
ctagtagcaactgcaaccggtgtacattcccaggtccagctggtacag

SEQ ID NO: 467 - DNA, 48 bp, Artificial Sequence
  Description of Artificial Sequence: Synthetic primer
ctagtagcaactgcaaccggtgtacattctgaggtgcagctggtggag

SEQ ID NO: 468 - DNA, 48 bp, Artificial Sequence
  Description of Artificial Sequence: Synthetic primer
ctagtagcaactgcaaccggtgtacattctcaggtgcagctggtggag

SEQ ID NO: 469 - DNA, 48 bp, Artificial Sequence
  Description of Artificial Sequence: Synthetic primer
ctagtagcaactgcaaccggtgtacattctgaggtgcagctgttggag

SEQ ID NO: 470 - DNA, 48 bp, Artificial Sequence
  Description of Artificial Sequence: Synthetic primer
ctagtagcaactgcaaccggtgtacattctgaagtgcagctggtggag

SEQ ID NO: 471 - DNA, 48 bp, Artificial Sequence
  Description of Artificial Sequence: Synthetic primer
ctagtagcaactgcaaccggtgtacattcccaggtgcagctgcaggag

SEQ ID NO: 472 - DNA, 50 bp, Artificial Sequence
  Description of Artificial Sequence: Synthetic primer
ctagtagcaactgcaaccggtgtacattcccaggtgcagctacagcagtg

SEQ ID NO: 473 - DNA, 48 bp, Artificial Sequence
  Description of Artificial Sequence: Synthetic primer
ctagtagcaactgcaaccggtgtacattcccagctgcagctgcaggag

SEQ ID NO: 474 - DNA, 48 bp, Artificial Sequence
  Description of Artificial Sequence: Synthetic primer
ctagtagcaactgcaaccggtgtacattcccaggtacagctgcagcag

SEQ ID NO: 475 - DNA, 40 bp, Artificial Sequence
  Description of Artificial Sequence: Synthetic primer
ccgatgggcccttggtcgacgctgaggagacggtgaccag

SEQ ID NO: 476 - DNA, 42 bp, Artificial Sequence
  Description of Artificial Sequence: Synthetic primer
ccgatgggcccttggtcgacgctgaagagacggtgaccattg

SEQ ID NO: 477 - DNA, 41 bp, Artificial Sequence
  Description of Artificial Sequence: Synthetic primer
ccgatgggcccttggtcgacgctgaggagacggtgaccgtg

SEQ ID NO: 478 - DNA, 20 bp, Artificial Sequence
  Description of Artificial Sequence: Synthetic primer
gtagcaactgcaaccggtgt

SEQ ID NO: 479 - DNA, 21 bp, Artificial Sequence
  Description of Artificial Sequence: Synthetic primer
gcttcgttagaacgcggctac

SEQ ID NO: 480 - DNA, 23 bp, Artificial Sequence
  Description of Artificial Sequence: Synthetic primer
ggaaggtgtgcacgccgctggtc

SEQ ID NO: 481 - DNA, 23 bp, Artificial Sequence
  Description of Artificial Sequence: Synthetic primer
ggtcctgggcccagtctgtgctg

SEQ ID NO: 482 - DNA, 23 bp, Artificial Sequence
  Description of Artificial Sequence: Synthetic primer
ggtcctgggcccagtctgccctg

SEQ ID NO: 483 - DNA, 23 bp, Artificial Sequence
  Description of Artificial Sequence: Synthetic primer
gctctgtgacctcctatgagctg

SEQ ID NO: 484 - DNA, 23 bp, Artificial Sequence
  Description of Artificial Sequence: Synthetic primer
ggtctctctcscagcytgtgctg

SEQ ID NO: 485 - DNA, 23 bp, Artificial Sequence
  Description of Artificial Sequence: Synthetic primer
gttcttgggccaattttatgctg

SEQ ID NO: 486 - DNA, 23 bp, Artificial Sequence
  Description of Artificial Sequence: Synthetic primer
ggtccaattcycaggctgtggtg

SEQ ID NO: 487 - DNA, 23 bp, Artificial Sequence
  Description of Artificial Sequence: Synthetic primer
gagtggattctcagactgtggtg

SEQ ID NO: 488 - DNA, 24 bp, Artificial Sequence
  Description of Artificial Sequence: Synthetic primer
caccagtgtggccttgttggcttg

SEQ ID NO: 489 - DNA, 48 bp, Artificial Sequence
  Description of Artificial Sequence: Synthetic primer
ctagtagcaactgcaaccggttcctgggcccagtctgtgctgackcag

SEQ ID NO: 490 - DNA, 48 bp, Artificial Sequence
  Description of Artificial Sequence: Synthetic primer
ctagtagcaactgcaaccggttcctgggcccagtctgccctgactcag

SEQ ID NO: 491 - DNA, 48 bp, Artificial Sequence
  Description of Artificial Sequence: Synthetic primer
ctagtagcaactgcaaccggttctgtgacctcctatgagctgacwcag

SEQ ID NO: 492 - DNA, 47 bp, Artificial Sequence
  Description of Artificial Sequence: Synthetic primer
ctagtagcaactgcaaccggttctctctcscagcytgtgctgactca

SEQ ID NO: 493 - DNA, 48 bp, Artificial Sequence
  Description of Artificial Sequence: Synthetic primer
ctagtagcaactgcaaccggttcttgggccaattttatgctgactcag

SEQ ID NO: 494 - DNA, 48 bp, Artificial Sequence
  Description of Artificial Sequence: Synthetic primer
ctagtagcaactgcaaccggttccaattcycagrctgtggtgacycag

SEQ ID NO: 495 - DNA, 37 bp, Artificial Sequence
  Description of Artificial Sequence: Synthetic primer
ggcttgaagctcctcactcgagggygggaacagagtg